European Patent Application EP 4 502 153 A1, published February 5, 2025. Title: GENE EDITING SYSTEM FOR TREATING USHER SYNDROME. Applicant: 주식회사 진코어. The sequence listing filed with the application follows.

SEQUENCE LISTING (545 sequences)

SEQ ID NO: 1 - DNA, 20 bp, Homo sapiens
  source 1..20: mol_type = genomic DNA; note = GK-USH2A-F02
cattcaagatagacgagaca

SEQ ID NO: 2 - DNA, 20 bp, Homo sapiens
  source 1..20: mol_type = genomic DNA; note = GK-USH2A-F03
tactgcagatgatacgaaca

SEQ ID NO: 3 - DNA, 20 bp, Homo sapiens
  source 1..20: mol_type = genomic DNA; note = GK-USH2A-F05
tagggggccaatcttactct

SEQ ID NO: 4 - DNA, 20 bp, Homo sapiens
  source 1..20: mol_type = genomic DNA; note = GK-USH2A-F06
gttgtatattaaagctaaat

SEQ ID NO: 5 - DNA, 20 bp, Homo sapiens
  source 1..20: mol_type = genomic DNA; note = GK-USH2A-F07
catcgcaaacagttgtatat

SEQ ID NO: 6 - DNA, 20 bp, Homo sapiens
  source 1..20: mol_type = genomic DNA; note = GK-USH2A-F09
ggagctctttttctctttaa

SEQ ID NO: 7 - DNA, 20 bp, Homo sapiens
  source 1..20: mol_type = genomic DNA; note = GK-USH2A-F10
ttttaacaaatgtgctcatt

SEQ ID NO: 8 - DNA, 20 bp, Homo sapiens
  source 1..20: mol_type = genomic DNA; note = GK-USH2A-F12
tactcagcttaaccttttat

SEQ ID NO: 9 - DNA, 22 bp, Homo sapiens
  source 1..22: mol_type = genomic DNA; note = GK-USH2A-F13
taataaaaggttaagctgagta

SEQ ID NO: 10 - DNA, 20 bp, Homo sapiens
  source 1..20: mol_type = genomic DNA; note = GK-USH2A-F15
gatcttaaatgttctcaccc

SEQ ID NO: 11 - DNA, 20 bp, Homo sapiens
  source 1..20: mol_type = genomic DNA; note = GK-USH2A-F16
tttgatatatgtacacatta

SEQ ID NO: 12 - DNA, 20 bp, Homo sapiens
  source 1..20: mol_type = genomic DNA; note = GK-USH2A-F17
cagcttcacgaaggtataat

SEQ ID NO: 13 - DNA, 20 bp, Homo sapiens
  source 1..20: mol_type = genomic DNA; note = GK-USH2A-F22
tcctttaaatagaagtaata

SEQ ID NO: 14 - DNA, 20 bp, Homo sapiens
  source 1..20: mol_type = genomic DNA; note = GK-USH2A-F23
tctgacaagtaaggttattc

SEQ ID NO: 15 - DNA, 20 bp, Homo sapiens
  source 1..20: mol_type = genomic DNA; note = GK-USH2A-F24
ggtattacaaggcaaagaaa

SEQ ID NO: 16 - DNA, 20 bp, Homo sapiens
  source 1..20: mol_type = genomic DNA; note = GK-USH2A-F25
gaatagtaaatgtttagatg

SEQ ID NO: 17 - DNA, 20 bp, Homo sapiens
  source 1..20: mol_type = genomic DNA; note = GK-USH2A-F26
taaaggaagtattttgcatc

SEQ ID NO: 18 - DNA, 20 bp, Homo sapiens
  source 1..20: mol_type = genomic DNA; note = GK-USH2A-F27
tacttcctttagatagtttc

SEQ ID NO: 19 - DNA, 20 bp, Homo sapiens
  source 1..20: mol_type = genomic DNA; note = GK-USH2A-F30
ttcaagctataattgcaatt

SEQ ID NO: 20 - DNA, 21 bp, Homo sapiens
  source 1..21: mol_type = genomic DNA; note = GK-USH2A-FA01
cattttcccatcctcaccttt

SEQ ID NO: 21 - DNA, 22 bp, Homo sapiens
  source 1..22: mol_type = genomic DNA; note = GK-USH2A-FA02
caactgtttgcgatgaacttca

SEQ ID NO: 22 - DNA, 20 bp, Homo sapiens
  source 1..20: mol_type = genomic DNA; note = GK-USH2A-FA03
tctttgcattaagtaataat

SEQ ID NO: 23 - DNA, 20 bp, Homo sapiens
  source 1..20: mol_type = genomic DNA; note = GK-USH2A-FA04
tttttaattattacttaatg

SEQ ID NO: 24 - DNA, 21 bp, Homo sapiens
  source 1..21: mol_type = genomic DNA; note = GK-USH2A-FA05
tatgtaattctactataattt

SEQ ID NO: 25 - DNA, 19 bp, Homo sapiens
  source 1..19: mol_type = genomic DNA; note = GK-USH2A-FA06
ttgctaagagattagatct

SEQ ID NO: 26 - DNA, 20 bp, Homo sapiens
  source 1..20: mol_type = genomic DNA; note = GK-USH2A-FA07
tttataatgtgtacatatat

SEQ ID NO: 27 - DNA, 22 bp, Homo sapiens
  source 1..22: mol_type = genomic DNA; note = GK-USH2A-FA08
caaaacatcatgttgtctgcca

SEQ ID NO: 28 - DNA, 21 bp, Homo sapiens
  source 1..21: mol_type = genomic DNA; note = GK-USH2A-FA09
cttcacgaaggtataattaaa

SEQ ID NO: 29 - DNA, 20 bp, Homo sapiens
  source 1..20: mol_type = genomic DNA; note = GK-USH2A-FA10
ggtgagtcattcatcactgt

SEQ ID NO: 30 - DNA, 20 bp, Homo sapiens
  source 1..20: mol_type = genomic DNA; note = GK-USH2A-FA11
tttattttccttattgaaat

SEQ ID NO: 31 - DNA, 20 bp, Homo sapiens
  source 1..20: mol_type = genomic DNA; note = GK-USH2A-FA12
tatatatgtatatatatgga

SEQ ID NO: 32 - DNA, 21 bp, Homo sapiens
  source 1..21: mol_type = genomic DNA; note = GK-USH2A-FA13
catatgtagaaaagcatttcc

SEQ ID NO: 33 - DNA, 20 bp, Homo sapiens
  source 1..20: mol_type = genomic DNA; note = GK-USH2A-FA14
tttaatttcaataaggaaaa

SEQ ID NO: 34 - DNA, 20 bp, Homo sapiens
  source 1..20: mol_type = genomic DNA; note = GK-USH2A-FA15
gttaacaatacagttatttt

SEQ ID NO: 35 - DNA, 20 bp, Homo sapiens
  source 1..20: mol_type = genomic DNA; note = GK-USH2A-FA16
gtagaccaattttaatagtt

SEQ ID NO: 36 - DNA, 20 bp, Homo sapiens
  source 1..20: mol_type = genomic DNA; note = GK-USH2A-FA17
gattcatatcatatcagttt

SEQ ID NO: 37 - DNA, 20 bp, Homo sapiens
  source 1..20: mol_type = genomic DNA; note = GK-USH2A-FA18
tatgactcattttgaactat

SEQ ID NO: 38 - DNA, 19 bp, Homo sapiens
  source 1..19: mol_type = genomic DNA; note = GK-USH2A-FA19
ccactattgctgcaaattt

SEQ ID NO: 39 - DNA, 19 bp, Homo sapiens
  source 1..19: mol_type = genomic DNA; note = GK-USH2A-FA20
ggaatatgtatggcatatt

SEQ ID NO: 40 - DNA, 19 bp, Homo sapiens
  source 1..19: mol_type = genomic DNA; note = GK-USH2A-FA21
taagcactgtgcatatttt

SEQ ID NO: 41 - DNA, 20 bp, Homo sapiens
  source 1..20: mol_type = genomic DNA; note = GK-USH2A-FA22
cttattttaagattaatttt

SEQ ID NO: 42 - DNA, 20 bp, Homo sapiens
  source 1..20: mol_type = genomic DNA; note = GK-USH2A-FA23
tttccaaatatccatgaatt

SEQ ID NO: 43 - DNA, 21 bp, Homo sapiens
  source 1..21: mol_type = genomic DNA; note = GK-USH2A-FA24
cagagatttaagtttaggtga

SEQ ID NO: 44 - DNA, 20 bp, Homo sapiens
  source 1..20: mol_type = genomic DNA; note = GK-USH2A-FA25
tgactcagaacatacctctt

SEQ ID NO: 45 - DNA, 20 bp, Homo sapiens
  source 1..20: mol_type = genomic DNA; note = GK-USH2A-FA26
tttatcattttcaattaata

SEQ ID NO: 46 - DNA, 20 bp, Homo sapiens
  source 1..20: mol_type = genomic DNA; note = GK-USH2A-FA27
tgataaaatagaggagcata

SEQ ID NO: 47 - DNA, 20 bp, Homo sapiens
  source 1..20: mol_type = genomic DNA; note = GK-USH2A-FA28
ttttatttatattaattact

SEQ ID NO: 48 - DNA, 21 bp, Homo sapiens
  source 1..21: mol_type = genomic DNA; note = GK-USH2A-FA29
taagtgtatatgctgttttca

SEQ ID NO: 49 - DNA, 21 bp, Homo sapiens
  source 1..21: mol_type = genomic DNA; note = GK-USH2A-FA30
catggatatttggaaactatc

SEQ ID NO: 50 - DNA, 20 bp, Homo sapiens
  source 1..20: mol_type = genomic DNA; note = GK-USH2A-R01
ggagaagttacctaagttaa

SEQ ID NO: 51 - DNA, 20 bp, Homo sapiens
  source 1..20: mol_type = genomic DNA; note = GK-USH2A-R02
gcttctacaaattttatttc

SEQ ID NO: 52 - DNA, 20 bp, Homo sapiens
  source 1..20: mol_type = genomic DNA; note = GK-USH2A-R04
ccgatcggctgagttttatc

SEQ ID NO: 53 - DNA, 20 bp, Homo sapiens
  source 1..20: mol_type = genomic DNA; note = GK-USH2A-R05
ctcaatttctacacttgaag

SEQ ID NO: 54 - DNA, 20 bp, Homo sapiens
  source 1..20: mol_type = genomic DNA; note = GK-USH2A-R07
cattgtatggatattcaact

SEQ ID NO: 55 - DNA, 20 bp, Homo sapiens
  source 1..20: mol_type = genomic DNA; note = GK-USH2A-R08
gttgaatatccatacaatgc

SEQ ID NO: 56 - DNA, 20 bp, Homo sapiens
  source 1..20: mol_type = genomic DNA; note = GK-USH2A-R09
tgatgaactaaatctctgaa

SEQ ID NO: 57 - DNA, 20 bp, Homo sapiens
  source 1..20: mol_type = genomic DNA; note = GK-USH2A-R10
caattctaggtatttctata

SEQ ID NO: 58 - DNA, 20 bp, Homo sapiens
  source 1..20: mol_type = genomic DNA; note = GK-USH2A-R11
gaattgtttccacatgccat

SEQ ID NO: 59 - DNA, 20 bp, Homo sapiens
  source 1..20: mol_type = genomic DNA; note = GK-USH2A-R13
tccacatgccatcaaattaa

SEQ ID NO: 60 - DNA, 20 bp, Homo sapiens
  source 1..20: mol_type = genomic DNA; note = GK-USH2A-R14
ctgtttaatctcattatata

SEQ ID NO: 61 - DNA, 20 bp, Homo sapiens
  source 1..20: mol_type = genomic DNA; note = GK-USH2A-R17
cttacatttaagattttaac

SEQ ID NO: 62 - DNA, 20 bp, Homo sapiens
  source 1..20: mol_type = genomic DNA; note = GK-USH2A-R18
ctctgagttatatgggtcta

SEQ ID NO: 63 - DNA, 20 bp, Homo sapiens
  source 1..20: mol_type = genomic DNA; note = GK-USH2A-R19
tctactccttctctggcaag

SEQ ID NO: 64 - DNA, 20 bp, Homo sapiens
  source 1..20: mol_type = genomic DNA; note = GK-USH2A-R20
ttgccagagaaggagtagaa

SEQ ID NO: 65 - DNA, 20 bp, Homo sapiens
  source 1..20: mol_type = genomic DNA; note = GK-USH2A-R22
tcttacacactgaccaatgc

SEQ ID NO: 66 - DNA, 20 bp, Homo sapiens
  source 1..20: mol_type = genomic DNA; note = GK-USH2A-R23
tctttttgtgatgtaagtat

SEQ ID NO: 67 - DNA, 20 bp, Homo sapiens
  source 1..20: mol_type = genomic DNA; note = GK-USH2A-R24
tattataactagatactcca

SEQ ID NO: 68 - DNA, 20 bp, Homo sapiens
  source 1..20: mol_type = genomic DNA; note = GK-USH2A-R26
tgtggctggtggtagaatta

SEQ ID NO: 69 - DNA, 20 bp, Homo sapiens
  source 1..20: mol_type = genomic DNA; note = GK-USH2A-R27
tataactaagaggtagctaa

SEQ ID NO: 70 - DNA, 20 bp, Homo sapiens
  source 1..20: mol_type = genomic DNA; note = GK-USH2A-R29
ctcagaggtaaccaaccaaa

SEQ ID NO: 71 - DNA, 20 bp, Homo sapiens
  source 1..20: mol_type = genomic DNA; note = GK-USH2A-R30
ttggctcagaggtaaccaac

SEQ ID NO: 72 - DNA, 20 bp, Homo sapiens
  source 1..20: mol_type = genomic DNA; note = GK-USH2A-R31
ccaggggtgtcacgtactta

SEQ ID NO: 73 - DNA, 20 bp, Homo sapiens
  source 1..20: mol_type = genomic DNA; note = GK-USH2A-R32
ctacctgatgaaatggtccc

SEQ ID NO: 74 - DNA, 20 bp, Homo sapiens
  source 1..20: mol_type = genomic DNA; note = GK-USH2A-R34
tgaaaggattaacctgaagg

SEQ ID NO: 75 - DNA, 20 bp, Homo sapiens
  source 1..20: mol_type = genomic DNA; note = GK-USH2A-R35
gagacaaaggactttgttgc

SEQ ID NO: 76 - DNA, 20 bp, Homo sapiens
  source 1..20: mol_type = genomic DNA; note = GK-USH2A-R36
tcctttgtctcctacacagt

SEQ ID NO: 77 - DNA, 20 bp, Homo sapiens
  source 1..20: mol_type = genomic DNA; note = GK-USH2A-R38
ttagatatctggtaggtgta

SEQ ID NO: 78 - DNA, 20 bp, Homo sapiens
  source 1..20: mol_type = genomic DNA; note = GK-USH2A-R39
gtcttatgcatggtgtagat

SEQ ID NO: 79 - DNA, 20 bp, Homo sapiens
  source 1..20: mol_type = genomic DNA; note = GK-USH2A-R40
tatacatccttctttctaag

SEQ ID NO: 80 - RNA, 20 nt, synthetic construct
  source 1..20: mol_type = other RNA; note = GUIDE-USH2A-F02
tgtctcgtctatcttgaatg

SEQ ID NO: 81 - RNA, 20 nt, synthetic construct
  source 1..20: mol_type = other RNA; note = GUIDE-USH2A-F03
tgttcgtatcatctgcagta

SEQ ID NO: 82 - RNA, 20 nt, synthetic construct
  source 1..20: mol_type = other RNA; note = GUIDE-USH2A-F05
agagtaagattggcccccta

SEQ ID NO: 83 - RNA, 20 nt, synthetic construct
  source 1..20: mol_type = other RNA; note = GUIDE-USH2A-F06
atttagctttaatatacaac

SEQ ID NO: 84 - RNA, 20 nt, synthetic construct
  source 1..20: mol_type = other RNA; note = GUIDE-USH2A-F07
atatacaactgtttgcgatg

SEQ ID NO: 85 - RNA, 20 nt, synthetic construct
  source 1..20: mol_type = other RNA; note = GUIDE-USH2A-F09
ttaaagagaaaaagagctcc

SEQ ID NO: 86 - RNA, 20 nt, synthetic construct
  source 1..20: mol_type = other RNA; note = GUIDE-USH2A-F10
aatgagcacatttgttaaaa

SEQ ID NO: 87 - RNA, 20 nt, synthetic construct
  source 1..20: mol_type = other RNA; note = GUIDE-USH2A-F12
ataaaaggttaagctgagta

SEQ ID NO: 88 - RNA, 22 nt, synthetic construct
  source 1..22: mol_type = other RNA; note = GUIDE-USH2A-F13
tactcagcttaaccttttatta

SEQ ID NO: 89 - RNA, 20 nt, synthetic construct
  source 1..20: mol_type = other RNA; note = GUIDE-USH2A-F15
gggtgagaacatttaagatc

SEQ ID NO: 90 - RNA, 20 nt, synthetic construct
  source 1..20: mol_type = other RNA; note = GUIDE-USH2A-F16
taatgtgtacatatatcaaa

SEQ ID NO: 91 - RNA, 20 nt, synthetic construct
  source 1..20: mol_type = other RNA; note = GUIDE-USH2A-F17
attataccttcgtgaagctg

SEQ ID NO: 92 - RNA, 20 nt, synthetic construct
  source 1..20: mol_type = other RNA; note = GUIDE-USH2A-F22
tattacttctatttaaagga

SEQ ID NO: 93 - RNA, 20 nt, synthetic construct
  source 1..20: mol_type = other RNA; note = GUIDE-USH2A-F23
gaataaccttacttgtcaga

SEQ ID NO: 94 - RNA, 20 nt, synthetic construct
  source 1..20: mol_type = other RNA; note = GUIDE-USH2A-F24
tttctttgccttgtaatacc

SEQ ID NO: 95 - RNA, 20 nt, synthetic construct
  source 1..20: mol_type = other RNA; note = GUIDE-USH2A-F25
catctaaacatttactattc

SEQ ID NO: 96 - RNA, 20 nt, synthetic construct
  source 1..20: mol_type = other RNA; note = GUIDE-USH2A-F26
gatgcaaaatacttccttta

SEQ ID NO: 97 - RNA, 20 nt, synthetic construct
  source 1..20: mol_type = other RNA; note = GUIDE-USH2A-F27
gaaactatctaaaggaagta

SEQ ID NO: 98 - RNA, 20 nt, synthetic construct
  source 1..20: mol_type = other RNA; note = GUIDE-USH2A-F30
aattgcaattatagcttgaa

SEQ ID NO: 99 - RNA, 21 nt, synthetic construct
  source 1..21: mol_type = other RNA; note = GUIDE-USH2A-FA01
aaaggtgaggatgggaaaatg

SEQ ID NO: 100 - RNA, 22 nt, synthetic construct
  source 1..22: mol_type = other RNA; note = GUIDE-USH2A-FA02
tgaagttcatcgcaaacagttg

SEQ ID NO: 101 - RNA, 20 nt, synthetic construct
  source 1..20: mol_type = other RNA; note = GUIDE-USH2A-FA03
attattacttaatgcaaaga

SEQ ID NO: 102 - RNA, 20 nt, synthetic construct
  source 1..20: mol_type = other RNA; note = GUIDE-USH2A-FA04
cattaagtaataattaaaaa

SEQ ID NO: 103 - RNA, 21 nt, synthetic construct
  source 1..21: mol_type = other RNA; note = GUIDE-USH2A-FA05
aaattatagtagaattacata

SEQ ID NO: 104 - RNA, 19 nt, synthetic construct
  source 1..19: mol_type = other RNA; note = GUIDE-USH2A-FA06
agatctaatctcttagcaa

SEQ ID NO: 105 - RNA, 20 nt, synthetic construct
  source 1..20: mol_type = other RNA; note = GUIDE-USH2A-FA07
atatatgtacacattataaa

SEQ ID NO: 106 - RNA, 22 nt, synthetic construct
  source 1..22: mol_type = other RNA; note = GUIDE-USH2A-FA08
tggcagacaacatgatgttttg

SEQ ID NO: 107 - RNA, 21 nt, synthetic construct
  source 1..21: mol_type = other RNA; note = GUIDE-USH2A-FA09
tttaattataccttcgtgaag

SEQ ID NO: 108 - RNA, 20 nt, synthetic construct
  source 1..20: mol_type = other RNA; note = GUIDE-USH2A-FA10
acagtgatgaatgactcacc

SEQ ID NO: 109 - RNA, 20 nt, synthetic construct
  source 1..20: mol_type = other RNA; note = GUIDE-USH2A-FA11
atttcaataaggaaaataaa

SEQ ID NO: 110 - RNA, 20 nt, synthetic construct
  source 1..20: mol_type = other RNA; note = GUIDE-USH2A-FA12
tccatatatatacatatata

SEQ ID NO: 111 - RNA, 21 nt, synthetic construct
  source 1..21: mol_type = other RNA; note = GUIDE-USH2A-FA13
ggaaatgcttttctacatatg

SEQ ID NO: 112 - RNA, 20 nt, synthetic construct
  source 1..20: mol_type = other RNA; note = GUIDE-USH2A-FA14
ttttccttattgaaattaaa

SEQ ID NO: 113 - RNA, 20 nt, synthetic construct
  source 1..20: mol_type = other RNA; note = GUIDE-USH2A-FA15
aaaataactgtattgttaac

SEQ ID NO: 114 - RNA, 20 nt, synthetic construct
  source 1..20: mol_type = other RNA; note = GUIDE-USH2A-FA16
aactattaaaattggtctac

SEQ ID NO: 115 - RNA, 20 nt, synthetic construct
  source 1..20: mol_type = other RNA; note = GUIDE-USH2A-FA17
aaactgatatgatatgaatc

SEQ ID NO: 116 - RNA, 20 nt, synthetic construct
  source 1..20: mol_type = other RNA; note = GUIDE-USH2A-FA18
atagttcaaaatgagtcata

SEQ ID NO: 117 - RNA, 19 nt, synthetic construct
  source 1..19: mol_type = other RNA; note = GUIDE-USH2A-FA19
aaatttgcagcaatagtgg

SEQ ID NO: 118 - RNA, 19 nt, synthetic construct
  source 1..19: mol_type = other RNA; note = GUIDE-USH2A-FA20
aatatgccatacatattcc

SEQ ID NO: 119 - RNA, 19 nt, synthetic construct
  source 1..19: mol_type = other RNA; note = GUIDE-USH2A-FA21
aaaatatgcacagtgctta

SEQ ID NO: 120 - RNA, 20 nt, synthetic construct
  source 1..20: mol_type = other RNA; note = GUIDE-USH2A-FA22
aaaattaatcttaaaataag

SEQ ID NO: 121 - RNA, 20 nt, synthetic construct
  source 1..20: mol_type = other RNA; note = GUIDE-USH2A-FA23
aattcatggatatttggaaa

SEQ ID NO: 122 - RNA, 21 nt, synthetic construct
  source 1..21: mol_type = other RNA; note = GUIDE-USH2A-FA24
tcacctaaacttaaatctctg

SEQ ID NO: 123 - RNA, 20 nt, synthetic construct
  source 1..20: mol_type = other RNA; note = GUIDE-USH2A-FA25
aagaggtatgttctgagtca

SEQ ID NO: 124 - RNA, 20 nt, synthetic construct
  source 1..20: mol_type = other RNA; note = GUIDE-USH2A-FA26
tattaattgaaaatgataaa

SEQ ID NO: 125 - RNA, 20 nt, synthetic construct
  source 1..20: mol_type = other RNA; note = GUIDE-USH2A-FA27
tatgctcctctattttatca

SEQ ID NO: 126 - RNA, 20 nt, synthetic construct
  source 1..20: mol_type = other RNA; note = GUIDE-USH2A-FA28
agtaattaatataaataaaa

SEQ ID NO: 127 - RNA, 21 nt, synthetic construct
  source 1..21: mol_type = other RNA; note = GUIDE-USH2A-FA29
tgaaaacagcatatacactta

SEQ ID NO: 128 - RNA, 21 nt, synthetic construct
  source 1..21: mol_type = other RNA; note = GUIDE-USH2A-FA30
gatagtttccaaatatccatg

SEQ ID NO: 129 - RNA, 20 nt, synthetic construct
  source 1..20: mol_type = other RNA; note = GUIDE-USH2A-R01
ttaacttaggtaacttctcc

SEQ ID NO: 130 - RNA, 20 nt, synthetic construct
  source 1..20: mol_type = other RNA; note = GUIDE-USH2A-R02
gaaataaaatttgtagaagc

SEQ ID NO: 131 - RNA, 20 nt, synthetic construct
  source 1..20: mol_type = other RNA; note = GUIDE-USH2A-R04
gataaaactcagccgatcgg

SEQ ID NO: 132 - RNA, 20 nt, synthetic construct
  source 1..20: mol_type = other RNA; note = GUIDE-USH2A-R05
cttcaagtgtagaaattgag

SEQ ID NO: 133 - RNA, 20 nt, synthetic construct
  source 1..20: mol_type = other RNA; note = GUIDE-USH2A-R07
agttgaatatccatacaatg

SEQ ID NO: 134 - RNA, 20 nt, synthetic construct
  source 1..20: mol_type = other RNA; note = GUIDE-USH2A-R08
gcattgtatggatattcaac

SEQ ID NO: 135 - RNA, 20 nt, synthetic construct
  source 1..20: mol_type = other RNA; note = GUIDE-USH2A-R09
ttcagagatttagttcatca

SEQ ID NO: 136 - RNA, 20 nt, synthetic construct
  source 1..20: mol_type = other RNA; note = GUIDE-USH2A-R10
tatagaaatacctagaattg

SEQ ID NO: 137 - RNA, 20 nt, synthetic construct
  source 1..20: mol_type = other RNA; note = GUIDE-USH2A-R11
atggcatgtggaaacaattc

SEQ ID NO: 138 - RNA, 20 nt, synthetic construct
  source 1..20: mol_type = other RNA; note = GUIDE-USH2A-R13
ttaatttgatggcatgtgga

SEQ ID NO: 139 - RNA, 20 nt, synthetic construct
  source 1..20: mol_type = other RNA; note = GUIDE-USH2A-R14
tatataatgagattaaacag

SEQ ID NO: 140 - RNA, 20 nt, synthetic construct
  source 1..20: mol_type = other RNA; note = GUIDE-USH2A-R17
gttaaaatcttaaatgtaag

SEQ ID NO: 141 - RNA, 20 nt, synthetic construct
  source 1..20: mol_type = other RNA; note = GUIDE-USH2A-R18
tagacccatataactcagag

SEQ ID NO: 142 - RNA, 20 nt, synthetic construct
  source 1..20: mol_type = other RNA; note = GUIDE-USH2A-R19
cttgccagagaaggagtaga

SEQ ID NO: 143 - RNA, 20 nt, synthetic construct
  source 1..20: mol_type = other RNA; note = GUIDE-USH2A-R20
ttctactccttctctggcaa

SEQ ID NO: 144 - RNA, 20 nt, synthetic construct
  source 1..20: mol_type = other RNA; note = GUIDE-USH2A-R22
gcattggtcagtgtgtaaga

SEQ ID NO: 145 - RNA, 20 nt, synthetic construct
  source 1..20: mol_type = other RNA; note = GUIDE-USH2A-R23
atacttacatcacaaaaaga

SEQ ID NO: 146 - RNA, 20 nt, synthetic construct
  source 1..20: mol_type = other RNA; note = GUIDE-USH2A-R24
tggagtatctagttataata

SEQ ID NO: 147 - RNA, 20 nt, synthetic construct
  source 1..20: mol_type = other RNA; note = GUIDE-USH2A-R26
taattctaccaccagccaca

SEQ ID NO: 148 - RNA, 20 nt, synthetic construct
  source 1..20: mol_type = other RNA; note = GUIDE-USH2A-R27
ttagctacctcttagttata

SEQ ID NO: 149 - RNA, 20 nt, synthetic construct
  source 1..20: mol_type = other RNA; note = GUIDE-USH2A-R29
tttggttggttacctctgag

SEQ ID NO: 150 - RNA, 20 nt, synthetic construct
  source 1..20: mol_type = other RNA; note = GUIDE-USH2A-R30
gttggttacctctgagccaa

SEQ ID NO: 151 - RNA, 20 nt, synthetic construct
  source 1..20: mol_type = other RNA; note = GUIDE-USH2A-R31
taagtacgtgacacccctgg

SEQ ID NO: 152 - RNA, 20 nt, synthetic construct
  source 1..20: mol_type = other RNA; note = GUIDE-USH2A-R32
gggaccatttcatcaggtag

SEQ ID NO: 153 - RNA, 20 nt, synthetic construct
  source 1..20: mol_type = other RNA; note = GUIDE-USH2A-R34
ccttcaggttaatcctttca

SEQ ID NO: 154 - RNA, 20 nt, synthetic construct
  source 1..20: mol_type = other RNA; note = GUIDE-USH2A-R35
gcaacaaagtcctttgtctc

SEQ ID NO: 155 - RNA, 20 nt, synthetic construct
  source 1..20: mol_type = other RNA; note = GUIDE-USH2A-R36
actgtgtaggagacaaagga

SEQ ID NO: 156 - RNA, 20 nt, synthetic construct
  source 1..20: mol_type = other RNA; note = GUIDE-USH2A-R38
tacacctaccagatatctaa

SEQ ID NO: 157 - RNA, 20 nt, synthetic construct
  source 1..20: mol_type = other RNA; note = GUIDE-USH2A-R39
atctacaccatgcataagac

SEQ ID NO: 158 - RNA, 20 nt, synthetic construct
  source 1..20: mol_type = other RNA; note = GUIDE-USH2A-R40
cttagaaagaaggatgtata

SEQ ID NO: 159 - RNA, 21 nt, synthetic construct
  source 1..21: mol_type = other RNA; note = GUIDE-USH2A-F16-21mer
taatgtgtacatatatcaaaa

SEQ ID NO: 160 - RNA, 22 nt, synthetic construct
  source 1..22: mol_type = other RNA; note = GUIDE-USH2A-F16-22mer
taatgtgtacatatatcaaaac

SEQ ID NO: 161 - RNA, 23 nt, synthetic construct
  source 1..23: mol_type = other RNA; note = GUIDE-USH2A-F16-23mer
taatgtgtacatatatcaaaaca

SEQ ID NO: 162 - RNA, 25 nt, synthetic construct
  source 1..25: mol_type = other RNA; note = GUIDE-USH2A-F16-25mer
taatgtgtacatatatcaaaacatc

SEQ ID NO: 163 - RNA, 23 nt, synthetic construct
  source 1..23: mol_type = other RNA; note = GUIDE-USH2A-FA12-23mer
tccatatatatacatatatatta

SEQ ID NO: 164 - RNA, 25 nt, synthetic construct
  source 1..25: mol_type = other RNA; note = GUIDE-USH2A-FA12-25mer
tccatatatatacatatatattatg

SEQ ID NO: 165 - RNA, 19 nt, synthetic construct
  source 1..19: mol_type = other RNA; note = GUIDE-USH2A-R19-19mer
cttgccagagaaggagtag

SEQ ID NO: 166 - RNA, 21 nt, synthetic construct
  source 1..21: mol_type = other RNA; note = GUIDE-USH2A-R19-21mer
cttgccagagaaggagtagaa

SEQ ID NO: 167 - RNA, 22 nt, synthetic construct
  source 1..22: mol_type = other RNA; note = GUIDE-USH2A-R19-22mer
cttgccagagaaggagtagaac

SEQ ID NO: 168 - RNA, 23 nt, synthetic construct
  source 1..23: mol_type = other RNA; note = GUIDE-USH2A-R19-23mer
cttgccagagaaggagtagaaca

SEQ ID NO: 169 - RNA, 24 nt, synthetic construct
  source 1..24: mol_type = other RNA; note = GUIDE-USH2A-R19-24mer
cttgccagagaaggagtagaacaa

SEQ ID NO: 170 - RNA, 25 nt, synthetic construct
  source 1..25: mol_type = other RNA; note = GUIDE-USH2A-R19-25mer
cttgccagagaaggagtagaacaaa

SEQ ID NO: 171 - RNA, 21 nt, synthetic construct
  source 1..21: mol_type = other RNA; note = GUIDE-USH2A-R40-21mer
cttagaaagaaggatgtataa

SEQ ID NO: 172 - RNA, 22 nt, synthetic construct
  source 1..22: mol_type = other RNA; note = GUIDE-USH2A-R40-22mer
cttagaaagaaggatgtataaa

SEQ ID NO: 173 - RNA, 24 nt, synthetic construct
  source 1..24: mol_type = other RNA; note = GUIDE-USH2A-R40-24mer
cttagaaagaaggatgtataaatc

SEQ ID NO: 174 - RNA, 25 nt, synthetic construct
  source 1..25: mol_type = other RNA; note = GUIDE-USH2A-R40-25mer
cttagaaagaaggatgtataaatca

SEQ ID NO: 175 - RNA, 161 nt, synthetic construct
  source 1..161: mol_type = other RNA; note = Wild-type tracrRNA of Cas12f1 gRNA
cttcactgataaagtggagaaccgcttcaccaaaagctgtcccttaggggattagaacttgagtgaaggtgggctgcttgcatcagcctaatgtcgagaagtgctttcttcggaaagtaaccctcgaaacaaattcatttttcctctccaattctgcacaa

SEQ ID NO: 176 - RNA, 37 nt, synthetic construct
  source 1..37: mol_type = other RNA; note = Wild-type crRNA of Cas12f1 gRNA
gttgcagaacccgaatagacgaatgaaggaatgcaac

SEQ ID NO: 177 - RNA, 222 nt, synthetic construct
  source 1..222: mol_type = other RNA; note = Canonical sgRNA for Cas12f1
  misc_feature 203..222: note = n is a, c, g or u
cttcactgataaagtggagaaccgcttcaccaaaagctgtcccttaggggattagaacttgagtgaaggtgggctgcttgcatcagcctaatgtcgagaagtgctttcttcggaaagtaaccctcgaaacaaattcatttttcctctccaattctgcacaagaaagttgcagaacccgaatagacgaatgaaggaatgcaacnnnnnnnnnnnnnnnnnnnn

SEQ ID NO: 178 - RNA, 20 nt, synthetic construct
  source 1..20: mol_type = other RNA; note = Xa of Formula (I)
cttcactgataaagtggaga

SEQ ID NO: 179 - RNA, 19 nt, synthetic construct
  source 1..19: mol_type = other RNA; note = Xa of Formula (I)
ttcactgataaagtggaga

SEQ ID NO: 180 - RNA, 18 nt, synthetic construct
  source 1..18: mol_type = other RNA; note = Xa of Formula (I)
tcactgataaagtggaga

SEQ ID NO: 181 - RNA, 17 nt, synthetic construct
  source 1..17: mol_type = other RNA; note = Xa of Formula (I)
cactgataaagtggaga

SEQ ID NO: 182 - RNA, 16 nt, synthetic construct
  source 1..16: mol_type = other RNA; note = Xa of Formula (I)
actgataaagtggaga

SEQ ID NO: 183 - RNA, 15 nt, synthetic construct
  source 1..15: mol_type = other RNA; note = Xa of Formula (I)
ctgataaagtggaga

SEQ ID NO: 184 - RNA, 14 nt, synthetic construct
  source 1..14: mol_type = other RNA; note = Xa of Formula (I)
tgataaagtggaga

SEQ ID NO: 185 - RNA, 13 nt, synthetic construct
  source 1..13: mol_type = other RNA; note = Xa of Formula (I)
gataaagtggaga

SEQ ID NO: 186 - RNA, 12 nt, synthetic construct
  source 1..12: mol_type = other RNA; note = Xa of Formula (I)
ataaagtggaga

SEQ ID NO: 187 - RNA, 11 nt, synthetic construct
  source 1..11: mol_type = other RNA; note = Xa of Formula (I)
taaagtggaga

SEQ ID NO: 188 - RNA, 10 nt, synthetic construct
  source 1..10: mol_type = other RNA; note = Xa of Formula (I)
aaagtggaga

SEQ ID NO: 189 - RNA, 13 nt, synthetic construct
  source 1..13: mol_type = other RNA; note = Xb1 of Formula (I)
caaaagctgtccc

SEQ ID NO: 190 - RNA, 12 nt, synthetic construct
  source 1..12: mol_type = other RNA; note = Xb1 of Formula (I)
caaaagctgtcc

SEQ ID NO: 191 - RNA, 11 nt, synthetic construct
  source 1..11: mol_type = other RNA; note = Xb1 of Formula (I)
caaaagctgtc

SEQ ID NO: 192 - RNA, 10 nt, synthetic construct
  source 1..10: mol_type = other RNA; note = Xb1 of Formula (I)
caaaagctgt

SEQ ID NO: 193 - RNA, 14 nt, synthetic construct
  source 1..14: mol_type = other RNA; note = Xb2 of Formula (I)
gggattagaacttg

SEQ ID NO: 194 - RNA, 13 nt, synthetic construct
  source 1..13: mol_type = other RNA; note = Xb2 of Formula (I)
ggattagaacttg

SEQ ID NO: 195 - RNA, 12 nt, synthetic construct
  source 1..12: mol_type = other RNA; note = Xb2 of Formula (I)
gattagaacttg

SEQ ID NO: 196 - RNA, 11 nt, synthetic construct
  source 1..11: mol_type = other RNA; note = Xb2 of Formula (I)
attagaacttg

SEQ ID NO: 197 - RNA, 10 nt, synthetic construct
  source 1..10: mol_type = other RNA; note = Xb2 of Formula (I)
ttagaacttg

SEQ ID NO: 198 - RNA, 31 nt, synthetic construct
  source 1..31: mol_type = other RNA; note = Xb1-UUAG-Xb2 of Formula (I)
caaaagctgtcccttaggggattagaacttg

SEQ ID NO: 199 - RNA, 25 nt, synthetic construct
  source 1..25: mol_type = other RNA; note = Xb1-UUAG-Xb2 of Formula (I)
caaaagctgtttagattagaacttg

SEQ ID NO: 200 - RNA, 20 nt, synthetic construct
  source 1..20: mol_type = other RNA; note = Xb1-UUAG-Xb2 of Formula (I)
caaaagctttagagaacttg

SEQ ID NO: 201 - RNA, 18 nt, synthetic construct
  source 1..18: mol_type = other RNA; note = Xb1-UUAG-Xb2 of Formula (I)
caaaagcttaggaacttg

SEQ ID NO: 202 - RNA, 10 nt, synthetic construct
  source 1..10: mol_type = other RNA; note = Xb1-UUAG-Xb2 of Formula (I)
caattagttg

SEQ ID NO: 203 - RNA, 28 nt, synthetic construct
  source 1..28: mol_type = other RNA; note = Xc1 of Formula (I)
ttcatttttcctctccaattctgcacaa

SEQ ID NO: 204 - RNA, 27 nt, synthetic construct
  source 1..27: mol_type = other RNA; note = Xc1 of Formula (I)
ttcatttttcctctccaattctgcaca

SEQ ID NO: 205 - RNA, 26 nt, synthetic construct
  source 1..26: mol_type = other RNA; note = Xc1 of Formula (I)
ttcatttttcctctccaattctgcac

SEQ ID NO: 206 - RNA, 25 nt, synthetic construct
  source 1..25: mol_type = other RNA; note = Xc1 of Formula (I)
ttcatttttcctctccaattctgca

SEQ ID NO: 207 - RNA, 24 nt, synthetic construct
  source 1..24: mol_type = other RNA; note = Xc1 of Formula (I)
ttcatttttcctctccaattctgc

SEQ ID NO: 208 - RNA, 23 nt, synthetic construct
  source 1..23: mol_type = other RNA; note = Xc1 of Formula (I)
ttcatttttcctctccaattctg

SEQ ID NO: 209 - RNA, 22 nt, synthetic construct
  source 1..22: mol_type = other RNA; note = Xc1 of Formula (I)
ttcatttttcctctccaattct

SEQ ID NO: 210 - RNA, 21 nt, synthetic construct
  source 1..21: mol_type = other RNA; note = Xc1 of Formula (I)
ttcatttttcctctccaattc

SEQ ID NO: 211 - RNA, 20 nt, synthetic construct
  source 1..20: mol_type = other RNA; note = Xc1 of Formula (I)
ttcatttttcctctccaatt

SEQ ID NO: 212 - RNA, 19 nt, synthetic construct
  source 1..19: mol_type = other RNA; note = Xc1 of Formula (I)
ttcatttttcctctccaat

SEQ ID NO: 213 - RNA, 18 nt, synthetic construct
  source 1..18: mol_type = other RNA; note = Xc1 of Formula (I)
ttcatttttcctctccaa

SEQ ID NO: 214 - RNA, 17 nt, synthetic construct
  source 1..17: mol_type = other RNA; note = Xc1 of Formula (I)
ttcatttttcctctcca

SEQ ID NO: 215 - RNA, 16 nt, synthetic construct
  source 1..16: mol_type = other RNA; note = Xc1 of Formula (I)
ttcatttttcctctcc

SEQ ID NO: 216 - RNA, 15 nt, synthetic construct
  source 1..15: mol_type = other RNA; note = Xc1 of Formula (I)
ttcatttttcctctc

SEQ ID NO: 217 - RNA, 14 nt, synthetic construct
  source 1..14: mol_type = other RNA; note = Xc1 of Formula (I)
ttcatttttcctct

SEQ ID NO: 218 - RNA, 13 nt, synthetic construct
  source 1..13: mol_type = other RNA; note = Xc1 of Formula (I)
ttcatttttcctc

SEQ ID NO: 219 - RNA, 12 nt, synthetic construct
  source 1..12: mol_type = other RNA; note = Xc1 of Formula (I)
ttcatttttcct

SEQ ID NO: 220 - RNA, 11 nt, synthetic construct
  source 1..11: mol_type = other RNA; note = Xc1 of Formula (I)
ttcatttttcc

SEQ ID NO: 221 - RNA, 10 nt, synthetic construct
  source 1..10: mol_type = other RNA; note = Xc1 of Formula (I)
ttcatttttc

SEQ ID NO: 222 - RNA, 27 nt, synthetic construct
  source 1..27: mol_type = other RNA; note = Xc2 of Formula (I)
gttgcagaacccgaatagacgaatgaa

SEQ ID NO: 223 - RNA, 26 nt, synthetic construct
  source 1..26: mol_type = other RNA; note = Xc2 of Formula (I)
ttgcagaacccgaatagacgaatgaa

SEQ ID NO: 224 - RNA, 25 nt, synthetic construct
  source 1..25: mol_type = other RNA; note = Xc2 of Formula (I)
tgcagaacccgaatagacgaatgaa

SEQ ID NO: 225 - RNA, 24 nt, synthetic construct
  source 1..24: mol_type = other RNA; note = Xc2 of Formula (I)
gcagaacccgaatagacgaatgaa

SEQ ID NO: 226 - RNA, 23 nt, synthetic construct
  source 1..23: mol_type = other RNA; note = Xc2 of Formula (I)
cagaacccgaatagacgaatgaa

SEQ ID NO: 227 - RNA, 22 nt, synthetic construct
  source 1..22: mol_type = other RNA; note = Xc2 of Formula (I)
agaacccgaatagacgaatgaa

SEQ ID NO: 228 - RNA, 21 nt, synthetic construct
  source 1..21: mol_type = other RNA; note = Xc2 of Formula (I)
gaacccgaatagacgaatgaa

SEQ ID NO: 229 - RNA, 20 nt, synthetic construct
  source 1..20: mol_type = other RNA; note = Xc2 of Formula (I)
aacccgaatagacgaatgaa

SEQ ID NO: 230 - RNA, 19 nt, synthetic construct
  source 1..19: mol_type = other RNA; note = Xc2 of Formula (I)
acccgaatagacgaatgaa

SEQ ID NO: 231 - RNA, 18 nt, synthetic construct
  source 1..18: mol_type = other RNA; note = Xc2 of Formula (I)
cccgaatagacgaatgaa

SEQ ID NO: 232 - RNA, 17 nt, synthetic construct
  source 1..17: mol_type = other RNA; note = Xc2 of Formula (I)
ccgaatagacgaatgaa

SEQ ID NO: 233 - RNA, 16 nt, synthetic construct
  source 1..16: mol_type = other RNA; note = Xc2 of Formula (I)
cgaatagacgaatgaa

SEQ ID NO: 234 - RNA, 15 nt, synthetic construct
  source 1..15: mol_type = other RNA; note = Xc2 of Formula (I)
gaatagacgaatgaa

SEQ ID NO: 235 - RNA, 14 nt, synthetic construct
  source 1..14: mol_type = other RNA; note = Xc2 of Formula (I)
aatagacgaatgaa

SEQ ID NO: 236 - RNA, 13 nt, synthetic construct
  source 1..13: mol_type = other RNA; note = Xc2 of Formula (I)
atagacgaatgaa

SEQ ID NO: 237 - RNA, 12 nt, synthetic construct
  source 1..12: mol_type = other RNA; note = Xc2 of Formula (I)
tagacgaatgaa

SEQ ID NO: 238 - RNA, 11 nt, synthetic construct
  source 1..11: mol_type = other RNA; note = Xc2 of Formula (I)
agacgaatgaa

SEQ ID NO: 239 - RNA, 10 nt, synthetic construct
  source 1..10: mol_type = other RNA; note = Xc2 of Formula (I)
gacgaatgaa

SEQ ID NO: 240 - RNA, 10 nt, synthetic construct
  source 1..10: mol_type = other RNA; note = Linker (Lk)
ttcgaaagaa

SEQ ID NO: 241 - RNA, 12 nt, synthetic construct
  source 1..12: mol_type = other RNA; note = Linker (Lk)
ttcagaaatgaa

SEQ ID NO: 242 - RNA, 14 nt, synthetic construct
  source 1..14: mol_type = other RNA; note = Linker (Lk)
ttcatgaaaatgaa

SEQ ID NO: 243 - RNA, 16 nt, synthetic construct
  source 1..16: mol_type = other RNA; note = Linker (Lk)
ttcattgaaaaatgaa

SEQ ID NO: 244 - RNA, 59 nt, synthetic construct
  source 1..59: mol_type = other RNA; note = Xc1-Lk-Xc2 of Formula (I)
ttcagtgctcctctccaattctgcacaagaaagttgcagaacccgaatagagcaatgaa

SEQ ID NO: 245 - RNA, 46 nt, synthetic construct
  source 1..46: mol_type = other RNA; note = Xc1-Lk-Xc2 of Formula (I)
ttcagtgctcctctccaattcgaaagaacccgaatagagcaatgaa

SEQ ID NO: 246 - RNA, 34 nt, synthetic construct
  source 1..34: mol_type = other RNA; note = Xc1-Lk-Xc2 of Formula (I)
ttcagtgctcctctcgaaagaatagagcaatgaa

SEQ ID NO: 247 - RNA, 22 nt, synthetic construct
  source 1..22: mol_type = other RNA; note = Xc1-Lk-Xc2 of Formula (I)
ttcagtgctgaaaagcaatgaa

SEQ ID NO: 248 - RNA, 18 nt, synthetic construct
  source 1..18: mol_type = other RNA; note = Xc1-Lk-Xc2 of Formula (I)
ttcatttgaaagaatgaa

SEQ ID NO: 249 - RNA, 14 nt, synthetic construct
  source 1..14: mol_type = other RNA; note = Xc1-Lk-Xc2 of Formula (I)
ttcatgaaaatgaa

SEQ ID NO: 250 - RNA, 10 nt, synthetic construct
  source 1..10: mol_type = other RNA; note = Xc1-Lk-Xc2 of Formula (I)
ttcgaaagaa

SEQ ID NO: 251 - RNA, 161 nt, synthetic construct
  source 1..161: mol_type = other RNA; note = Engineered tracrRNA (MS1)
cttcactgataaagtggagaaccgcttcaccaaaagctgtcccttaggggattagaacttgagtgaaggtgggctgcttgcatcagcctaatgtcgagaagtgctttcttcggaaagtaaccctcgaaacaaattcagtgctcctctccaattctgcacaa

SEQ ID NO: 252 - RNA, 154 nt, synthetic construct
  source 1..154: mol_type = other RNA; note = Engineered tracrRNA (MS1/MS3-1)
gataaagtggagaaccgcttcaccaaaagctgtcccttaggggattagaacttgagtgaaggtgggctgcttgcatcagcctaatgtcgagaagtgctttcttcggaaagtaaccctcgaaacaaattcagtgctcctctccaattctgcacaa

SEQ ID NO: 253 - RNA, 147 nt, synthetic construct
  source 1..147: mol_type = other RNA; note = Engineered tracrRNA (MS1/MS3-2)
tggagaaccgcttcaccaaaagctgtcccttaggggattagaacttgagtgaaggtgggctgcttgcatcagcctaatgtcgagaagtgctttcttcggaaagtaaccctcgaaacaaattcagtgctcctctccaattctgcacaa

SEQ ID NO: 254 - RNA, 141 nt, synthetic construct
  source 1..141: mol_type = other RNA; note = Engineered tracrRNA (MS1/MS3-3)
accgcttcaccaaaagctgtcccttaggggattagaacttgagtgaaggtgggctgcttgcatcagcctaatgtcgagaagtgctttcttcggaaagtaaccctcgaaacaaattcagtgctcctctccaattctgcacaa

SEQ ID NO: 255 - RNA, 154 nt, synthetic construct
  source 1..154: mol_type = other RNA; note = Engineered tracrRNA (MS1/MS4*-1)
cttcactgataaagtggagaaccgcttcaccaaaagctgtcccttaggggattagaacttgagtgaaggtgggctgcttgcatcagcctaatgtcgagaagtgctttcttcggaaagtaaccctcgaaacaaattcagtgctcctctccaattc

SEQ ID NO: 256 - RNA, 148 nt, synthetic construct
  source 1..148: mol_type = other RNA; note = Engineered tracrRNA (MS1/MS4*-2)
cttcactgataaagtggagaaccgcttcaccaaaagctgtcccttaggggattagaacttgagtgaaggtgggctgcttgcatcagcctaatgtcgagaagtgctttcttcggaaagtaaccctcgaaacaaattcagtgctcctctc

SEQ ID NO: 257 - RNA, 142 nt, synthetic construct
  source 1..142: mol_type = other RNA; note = Engineered tracrRNA (MS1/MS4*-3)
cttcactgataaagtggagaaccgcttcaccaaaagctgtcccttaggggattagaacttgagtgaaggtgggctgcttgcatcagcctaatgtcgagaagtgctttcttcggaaagtaaccctcgaaacaaattcagtgct

SEQ ID NO: 258 - RNA, 155 nt, synthetic construct
  source 1..155: mol_type = other RNA; note = Engineered tracrRNA (MS1/MS5-1)
cttcactgataaagtggagaaccgcttcaccaaaagctgtttagattagaacttgagtgaaggtgggctgcttgcatcagcctaatgtcgagaagtgctttcttcggaaagtaaccctcgaaacaaattcagtgctcctctccaattctgcacaa

SEQ ID NO: 259 - RNA, 148 nt, synthetic construct
  source 1..148: mol_type = other RNA; note = Engineered tracrRNA (MS1/MS5-2)
cttcactgataaagtggagaaccgcttcaccaaaagcttaggaacttgagtgaaggtgggctgcttgcatcagcctaatgtcgagaagtgctttcttcggaaagtaaccctcgaaacaaattcagtgctcctctccaattctgcacaa

SEQ ID NO: 260 - RNA, 140 nt, synthetic construct
  source 1..140: mol_type = other RNA; note = Engineered tracrRNA (MS1/MS5-3)
cttcactgataaagtggagaaccgcttcaccaattagttgagtgaaggtgggctgcttgcatcagcctaatgtcgagaagtgctttcttcggaaagtaaccctcgaaacaaattcagtgctcctctccaattctgcacaa

SEQ ID NO: 261 - RNA, 134 nt, synthetic construct
  source 1..134: mol_type = other RNA; note = Engineered tracrRNA (MS1/MS3-3/MS4*-1)
accgcttcaccaaaagctgtcccttaggggattagaacttgagtgaaggtgggctgcttgcatcagcctaatgtcgagaagtgctttcttcggaaagtaaccctcgaaacaaattcagtgctcctctccaattc

SEQ ID NO: 262 - RNA, 128 nt, synthetic construct
  source 1..128: mol_type = other RNA; note = Engineered tracrRNA (MS1/MS3-3/MS4*-2)
accgcttcaccaaaagctgtcccttaggggattagaacttgagtgaaggtgggctgcttgcatcagcctaatgtcgagaagtgctttcttcggaaagtaaccctcgaaacaaattcagtgctcctctc

SEQ ID NO: 263 - RNA, 122 nt, synthetic construct
  source 1..122: mol_type = other RNA; note = Engineered tracrRNA (MS1/MS3-3/MS4*-3)
accgcttcaccaaaagctgtcccttaggggattagaacttgagtgaaggtgggctgcttgcatcagcctaatgtcgagaagtgctttcttcggaaagtaaccctcgaaacaaattcagtgct

SEQ ID NO: 264 - RNA, 142 nt, synthetic construct
  source 1..142: mol_type = other RNA; note = Engineered tracrRNA (MS1/MS4*-2/MS5-1)
cttcactgataaagtggagaaccgcttcaccaaaagctgtttagattagaacttgagtgaaggtgggctgcttgcatcagcctaatgtcgagaagtgctttcttcggaaagtaaccctcgaaacaaattcagtgctcctctc

SEQ ID NO: 265 - RNA, 135 nt, synthetic construct
  source 1..135: mol_type = other RNA; note = Engineered tracrRNA (MS1/MS4*-2/MS5-2)
cttcactgataaagtggagaaccgcttcaccaaaagcttaggaacttgagtgaaggtgggctgcttgcatcagcctaatgtcgagaagtgctttcttcggaaagtaaccctcgaaacaaattcagtgctcctctc

SEQ ID NO: 266 - RNA, 127 nt, synthetic construct
  source 1..127: mol_type = other RNA; note = Engineered tracrRNA (MS1/MS4*-2/MS5-3)
cttcactgataaagtggagaaccgcttcaccaattagttgagtgaaggtgggctgcttgcatcagcctaatgtcgagaagtgctttcttcggaaagtaaccctcgaaacaaattcagtgctcctctc

SEQ ID NO: 267 - RNA, 135 nt, synthetic construct
  source 1..135: mol_type = other RNA; note = Engineered tracrRNA (MS1/MS3-3/MS5-1)
accgcttcaccaaaagctgtttagattagaacttgagtgaaggtgggctgcttgcatcagcctaatgtcgagaagtgctttcttcggaaagtaaccctcgaaacaaattcagtgctcctctccaattctgcacaa

SEQ ID NO: 268 - RNA, 128 nt, synthetic construct
  source 1..128: mol_type = other RNA; note = Engineered tracrRNA (MS1/MS3-3/MS5-2)
accgcttcaccaaaagcttaggaacttgagtgaaggtgggctgcttgcatcagcctaatgtcgagaagtgctttcttcggaaagtaaccctcgaaacaaattcagtgctcctctccaattctgcacaa

SEQ ID NO: 269 - RNA, 120 nt, synthetic construct
  source 1..120: mol_type = other RNA; note = Engineered tracrRNA (MS1/MS3-3/MS5-3)
accgcttcaccaattagttgagtgaaggtgggctgcttgcatcagcctaatgtcgagaagtgctttcttcggaaagtaaccctcgaaacaaattcagtgctcctctccaattctgcacaa

SEQ ID NO: 270 - RNA, 107 nt, synthetic construct
  source 1..107: mol_type = other RNA; note = Engineered tracrRNA (MS1/MS3-3/MS4*-2/MS5-3)
accgcttcaccaattagttgagtgaaggtgggctgcttgcatcagcctaatgtcgagaagtgctttcttcggaaagtaaccctcgaaacaaattcagtgctcctctc

SEQ ID NO: 271 - RNA, 140 nt, synthetic construct
  source 1..140: mol_type = other RNA; note = Engineered tracrRNA (MF)
cttcactgataaagtggagaaccgcttcaccaaaagctgtcccttaggggattagaacttgagtgaaggtgggctgcttgcatcagcctaatgtcgagaagtgctttcttcggaaagtaaccctcgaaacaaattcattt

SEQ ID NO: 272 - RNA, 133 nt, synthetic construct
  source 1..133: mol_type = other RNA; note = Engineered tracrRNA (MF/MS3-1)
gataaagtggagaaccgcttcaccaaaagctgtcccttaggggattagaacttgagtgaaggtgggctgcttgcatcagcctaatgtcgagaagtgctttcttcggaaagtaaccctcgaaacaaattcattt

SEQ ID NO: 273 - RNA, 126 nt, synthetic construct
  source 1..126: mol_type = other RNA; note = Engineered tracrRNA (MF/MS3-2)
tggagaaccgcttcaccaaaagctgtcccttaggggattagaacttgagtgaaggtgggctgcttgcatcagcctaatgtcgagaagtgctttcttcggaaagtaaccctcgaaacaaattcattt

SEQ ID NO: 274 - RNA, 120 nt, synthetic construct
  source 1..120: mol_type = other RNA; note = Engineered tracrRNA (MF/MS3-3)
accgcttcaccaaaagctgtcccttaggggattagaacttgagtgaaggtgggctgcttgcatcagcctaatgtcgagaagtgctttcttcggaaagtaaccctcgaaacaaattcattt

SEQ ID NO: 275 - RNA, 138 nt, synthetic construct
  source 1..138: mol_type = other RNA; note = Engineered tracrRNA (MF/MS4-1)
cttcactgataaagtggagaaccgcttcaccaaaagctgtcccttaggggattagaacttgagtgaaggtgggctgcttgcatcagcctaatgtcgagaagtgctttcttcggaaagtaaccctcgaaacaaattcat

SEQ ID NO: 276 - RNA, 136 nt, synthetic construct
  source 1..136: mol_type = other RNA; note = Engineered tracrRNA (MF/MS4-2)
cttcactgataaagtggagaaccgcttcaccaaaagctgtcccttaggggattagaacttgagtgaaggtgggctgcttgcatcagcctaatgtcgagaagtgctttcttcggaaagtaaccctcgaaacaaattc

SEQ ID NO: 277 - RNA, 133 nt, synthetic construct
  source 1..133: mol_type = other RNA; note = Engineered tracrRNA (MF/MS4-3)
cttcactgataaagtggagaaccgcttcaccaaaagctgtcccttaggggattagaacttgagtgaaggtgggctgcttgcatcagcctaatgtcgagaagtgctttcttcggaaagtaaccctcgaaacaaa

SEQ ID NO: 278 - RNA, 134 nt, synthetic construct
  source 1..134: mol_type = other RNA; note = Engineered tracrRNA (MF/MS5-1)
cttcactgataaagtggagaaccgcttcaccaaaagctgtttagattagaacttgagtgaaggtgggctgcttgcatcagcctaatgtcgagaagtgctttcttcggaaagtaaccctcgaaacaaattcattt

SEQ ID NO: 279 - RNA, 129 nt, synthetic construct
  source 1..129: mol_type = other RNA; note = Engineered tracrRNA (MF/MS5-2)
cttcactgataaagtggagaaccgcttcaccaaaagctttagagaacttgagtgaaggtgggctgcttgcatcagcctaatgtcgagaagtgctttcttcggaaagtaaccctcgaaacaaattcattt

SEQ ID NO: 280 - RNA, 119 nt, synthetic construct
  source 1..119: mol_type = other RNA; note = Engineered tracrRNA (MF/MS5-3)
cttcactgataaagtggagaaccgcttcaccaattagttgagtgaaggtgggctgcttgcatcagcctaatgtcgagaagtgctttcttcggaaagtaaccctcgaaacaaattcattt

SEQ ID NO: 281 - RNA, 113 nt, synthetic construct
  source 1..113: mol_type = other RNA; note = Engineered tracrRNA (MF/MS5)
cttcactgataaagtggagaaccgcttcacttagagtgaaggtgggctgcttgcatcagcctaatgtcgagaagtgctttcttcggaaagtaaccctcgaaacaaattcattt

SEQ ID NO: 282 - RNA, 118 nt, synthetic construct
  source 1..118: mol_type = other RNA; note = Engineered tracrRNA (MF/MS3-3/MS4-1)
accgcttcaccaaaagctgtcccttaggggattagaacttgagtgaaggtgggctgcttgcatcagcctaatgtcgagaagtgctttcttcggaaagtaaccctcgaaacaaattcat

SEQ ID NO: 283 - RNA, 116 nt, synthetic construct
  source 1..116: mol_type = other RNA; note = Engineered tracrRNA (MF/MS3-3/MS4-2)
accgcttcaccaaaagctgtcccttaggggattagaacttgagtgaaggtgggctgcttgcatcagcctaatgtcgagaagtgctttcttcggaaagtaaccctcgaaacaaattc

SEQ ID NO: 284 - RNA, 113 nt, synthetic construct
  source 1..113: mol_type = other RNA; note = Engineered tracrRNA (MF/MS3-3/MS4-3)
accgcttcaccaaaagctgtcccttaggggattagaacttgagtgaaggtgggctgcttgcatcagcctaatgtcgagaagtgctttcttcggaaagtaaccctcgaaacaaa

SEQ ID NO: 285 - RNA, 127 nt, synthetic construct
  source 1..127: mol_type = other RNA; note = Engineered tracrRNA (MF/MS4-3/MS5-1)
cttcactgataaagtggagaaccgcttcaccaaaagctgtttagattagaacttgagtgaaggtgggctgcttgcatcagcctaatgtcgagaagtgctttcttcggaaagtaaccctcgaaacaaa

SEQ ID NO: 286 - RNA, 122 nt, synthetic construct
  source 1..122: mol_type = other RNA; note = Engineered tracrRNA (MF/MS4-3/MS5-2)
cttcactgataaagtggagaaccgcttcaccaaaagctttagagaacttgagtgaaggtgggctgcttgcatcagcctaatgtcgagaagtgctttcttcggaaagtaaccctcgaaacaaa

SEQ ID NO: 287 - RNA, 112 nt, synthetic construct
  source 1..112: mol_type = other RNA; note = Engineered tracrRNA (MF/MS4-3/MS5-3)
cttcactgataaagtggagaaccgcttcaccaattagttgagtgaaggtgggctgcttgcatcagcctaatgtcgagaagtgctttcttcggaaagtaaccctcgaaacaaa

SEQ ID NO: 288 - RNA, 106 nt, synthetic construct
  source 1..106: mol_type = other RNA; note = Engineered tracrRNA (MF/MS4-3/MS5)
cttcactgataaagtggagaaccgcttcacttagagtgaaggtgggctgcttgcatcagcctaatgtcgagaagtgctttcttcggaaagtaaccctcgaaacaaa

SEQ ID NO: 289 - RNA, 114 nt, synthetic construct
  source 1..114: mol_type = other RNA; note = Engineered tracrRNA (MF/MS3-3/MS5-1)
accgcttcaccaaaagctgtttagattagaacttgagtgaaggtgggctgcttgcatcagcctaatgtcgagaagtgctttcttcggaaagtaaccctcgaaacaaattcattt

SEQ ID NO: 290 - RNA, 109 nt, synthetic construct
  source 1..109: mol_type = other RNA; note = Engineered tracrRNA (MF/MS3-3/MS5-2)
accgcttcaccaaaagctttagagaacttgagtgaaggtgggctgcttgcatcagcctaatgtcgagaagtgctttcttcggaaagtaaccctcgaaacaaattcattt

SEQ ID NO: 291 - RNA, 99 nt, synthetic construct
  source 1..99: mol_type = other RNA; note = Engineered tracrRNA (MF/MS3-3/MS5-3)
accgcttcaccaattagttgagtgaaggtgggctgcttgcatcagcctaatgtcgagaagtgctttcttcggaaagtaaccctcgaaacaaattcattt

SEQ ID NO: 292 - RNA, 93 nt, synthetic construct
  source 1..93: mol_type = other RNA; note = Engineered tracrRNA (MF/MS3-3/MS5)
accgcttcacttagagtgaaggtgggctgcttgcatcagcctaatgtcgagaagtgctttcttcggaaagtaaccctcgaaacaaattcattt

SEQ ID NO: 293 - RNA, 92 nt, synthetic construct
  source 1..92: mol_type = other RNA; note = Engineered tracrRNA (MF/MS3-3/MS4-3/MS5-3)
accgcttcaccaattagttgagtgaaggtgggctgcttgcatcagcctaatgtcgagaagtgctttcttcggaaagtaaccctcgaaacaaa

SEQ ID NO: 294 - RNA, 91 nt, synthetic construct
  source 1..91: mol_type = other RNA; note = Engineered tracrRNA (MF/MS3-3/MS4-1/MS5)
accgcttcacttagagtgaaggtgggctgcttgcatcagcctaatgtcgagaagtgctttcttcggaaagtaaccctcgaaacaaattcat

SEQ ID NO: 295 - RNA, 89 nt, synthetic construct
  source 1..89: mol_type = other RNA; note = Engineered tracrRNA (MF/MS3-3/MS4-2/MS5)
accgcttcacttagagtgaaggtgggctgcttgcatcagcctaatgtcgagaagtgctttcttcggaaagtaaccctcgaaacaaattc

SEQ ID NO: 296 - RNA, 86 nt, synthetic construct
  source 1..86: mol_type = other RNA; note = Engineered tracrRNA (MF/MS3-3/MS4-3/MS5)
accgcttcacttagagtgaaggtgggctgcttgcatcagcctaatgtcgagaagtgctttcttcggaaagtaaccctcgaaacaaa

SEQ ID NO: 297 - RNA, 37 nt, synthetic construct
  source 1..37: mol_type = other RNA; note = Engineered crRNA (MS1)
gttgcagaacccgaatagagcaatgaaggaatgcaac

SEQ ID NO: 298 - RNA, 31 nt, synthetic construct
  source 1..31: mol_type = other RNA; note = Engineered crRNA (MS1/MS4*-1)
gaacccgaatagagcaatgaaggaatgcaac

SEQ ID NO: 299 - RNA, 25 nt, synthetic construct
  source 1..25: mol_type = other RNA; note = Engineered crRNA (MS1/MS4*-2)
gaatagagcaatgaaggaatgcaac

SEQ ID NO: 300 - RNA, 19 nt, synthetic construct
  source 1..19: mol_type = other RNA; note = Engineered crRNA (MS1/MS4*-3)
agcaatgaaggaatgcaac

SEQ ID NO: 301 - RNA, 17 nt, synthetic construct
  source 1..17: mol_type = other RNA; note = Engineered crRNA (MF)
gaatgaaggaatgcaac

SEQ ID NO: 302 - RNA, 15 nt, synthetic construct
  source 1..15: mol_type = other RNA; note = Engineered crRNA (MF/MS4-1)
atgaaggaatgcaac

SEQ ID NO: 303 - RNA, 13 nt, synthetic construct
  source 1..13: mol_type = other RNA; note = Engineered crRNA (MF/MS4-2)
gaaggaatgcaac

SEQ ID NO: 304 - RNA, 10 nt, synthetic construct
  source 1..10: mol_type = other RNA; note = Engineered crRNA (MF/MS4-3)
ggaatgcaac

SEQ ID NO: 305 - RNA, 68 nt, synthetic construct
  source 1..68: mol_type = other RNA; note = Engineered crRNA (MS1/MS2)
  misc_feature 38..57: note = n is a, c, g or u
gttgcagaacccgaatagagcaatgaaggaatgcaacnnnnnnnnnnnnnnnnnnnnttttatttttt

SEQ ID NO: 306 - RNA, 62 nt, synthetic construct
  source 1..62: mol_type = other RNA; note = Engineered crRNA (MS1/MS2/MS4*-1)
  misc_feature 32..51: note = n is a, c, g or u
gaacccgaatagagcaatgaaggaatgcaacnnnnnnnnnnnnnnnnnnnnttttatttttt

SEQ ID NO: 307 - RNA, 56 nt, synthetic construct
  source 1..56: mol_type = other RNA; note = Engineered crRNA (MS1/MS2/MS4*-2)
  misc_feature 26..45: note = n is a, c, g or u
gaatagagcaatgaaggaatgcaacnnnnnnnnnnnnnnnnnnnnttttatttttt

SEQ ID NO: 308 - RNA, 50 nt, synthetic construct
  source 1..50: mol_type = other RNA; note = Engineered crRNA (MS1/MS2/MS4*-3)
  misc_feature 20..39: note = n is a, c, g or u
agcaatgaaggaatgcaacnnnnnnnnnnnnnnnnnnnnttttatttttt

SEQ ID NO: 309 - RNA, 48 nt, synthetic construct
  source 1..48: mol_type = other RNA; note = Engineered crRNA (MF/MS2)
  misc_feature 18..37: note = n is a, c, g or u
gaatgaaggaatgcaacnnnnnnnnnnnnnnnnnnnnttttatttttt

SEQ ID NO: 310 - RNA, 46 nt, synthetic construct
  source 1..46: mol_type = other RNA; note = Engineered crRNA (MF/MS2/MS4-1)
  misc_feature 16..35: note = n is a, c, g or u
atgaaggaatgcaacnnnnnnnnnnnnnnnnnnnnttttatttttt

SEQ ID NO: 311 - RNA, 44 nt, synthetic construct
  source 1..44: mol_type = other RNA; note = Engineered crRNA (MF/MS2/MS4-2)
  misc_feature 14..33: note = n is a, c, g or u
gaaggaatgcaacnnnnnnnnnnnnnnnnnnnnttttatttttt

SEQ ID NO: 312 - RNA, 41 nt, synthetic construct
  source 1..41: mol_type = other RNA; note = Engineered crRNA (MF/MS2/MS4-3)
  misc_feature 11..30: note = n is a, c, g or u
ggaatgcaacnnnnnnnnnnnnnnnnnnnnttttatttttt

SEQ ID NO: 313 - RNA, 222 nt, synthetic construct
  source 1..222: mol_type = other RNA; note = Engineered sgRNA with modification of MS1
  misc_feature 203..222: note = n is a, c, g or u
cttcactgataaagtggagaaccgcttcaccaaaagctgtcccttaggggattagaacttgagtgaaggtgggctgcttgcatcagcctaatgtcgagaagtgctttcttcggaaagtaaccctcgaaacaaattcagtgctcctctccaattctgcacaagaaagttgcagaacccgaatagagcaatgaaggaatgcaacnnnnnnnnnnnnnnnnnnnn

SEQ ID NO: 314 - RNA, 233 nt, synthetic construct
  source 1..233: mol_type = other RNA; note = Engineered sgRNA with modification of MS1/MS2
  misc_feature 203..222: note = n is a, c, g or u
cttcactgataaagtggagaaccgcttcaccaaaagctgtcccttaggggattagaacttgagtgaaggtgggctgcttgcatcagcctaatgtcgagaagtgctttcttcggaaagtaaccctcgaaacaaattcagtgctcctctccaattctgcacaagaaagttgcagaacccgaatagagcaatgaaggaatgcaacnnnnnnnnnnnnnnnnnnnnttttatttttt

SEQ ID NO: 315 - RNA, 213 nt, synthetic construct
  source 1..213: mol_type = other RNA; note = Engineered sgRNA with modification of MS1/MS2/MS3
  misc_structure 183..202: note = n is a, c, g or u
accgcttcaccaaaagctgtcccttaggggattagaacttgagtgaaggtgggctgcttgcatcagcctaatgtcgagaagtgctttcttcggaaagtaaccctcgaaacaaattcagtgctcctctccaattctgcacaagaaagttgcagaacccgaatagagcaatgaaggaatgcaacnnnnnnnnnnnnnnnnnnnnttttatttttt

SEQ ID NO: 316 - RNA, 158 nt, synthetic construct
  source 1..158: mol_type = other RNA; note = Engineered sgRNA with modification of MS2/MS3/MS4
  misc_feature 128..147: note = n is a, c, g or u
accgcttcaccaaaagctgtcccttaggggattagaacttgagtgaaggtgggctgcttgcatcagcctaatgtcgagaagtgctttcttcggaaagtaaccctcgaaacaaagaaaggaatgcaacnnnnnnnnnnnnnnnnnnnnttttatttttt

SEQ ID NO: 317 - RNA, 131 nt, synthetic construct
  source 1..131: mol_type = other RNA; note = Engineered sgRNA with modification of MS2/MS3/MS4/MS5
  misc_feature 99..118: note = n is a, c, g or u
accgcttcacttagagtgaaggtgggctgcttgcatcagcctaatgtcgagaagtgctttcttcggaaagtaaccctcgaaacaaagaaaggaatgcaacnnnnnnnnnnnnnnnnnnnnttttatttttt

SEQ ID NO: 318 - RNA, 215 nt, synthetic construct
  source 1..215: mol_type = other RNA; note = Engineered sgRNA with modification of MS1/MS3-1
  misc_feature 196..215: note = n is a, c, g or u
gataaagtggagaaccgcttcaccaaaagctgtcccttaggggattagaacttgagtgaaggtgggctgcttgcatcagcctaatgtcgagaagtgctttcttcggaaagtaaccctcgaaacaaattcagtgctcctctccaattctgcacaagaaagttgcagaacccgaatagagcaatgaaggaatgcaacnnnnnnnnnnnnnnnnnnnn

SEQ ID NO: 319 - RNA, 208 nt, synthetic construct
  source 1..208: mol_type = other RNA; note = Engineered sgRNA with modification of MS1/MS3-2
  misc_feature 189..208: note = n is a, c, g or u
tggagaaccgcttcaccaaaagctgtcccttaggggattagaacttgagtgaaggtgggctgcttgcatcagcctaatgtcgagaagtgctttcttcggaaagtaaccctcgaaacaaattcagtgctcctctccaattctgcacaagaaagttgcagaacccgaatagagcaatgaaggaatgcaacnnnnnnnnnnnnnnnnnnnn

SEQ ID NO: 320 - RNA, 202 nt, synthetic construct
  source 1..202: mol_type = other RNA; note = Engineered sgRNA with modification of MS1/MS3-3
  misc_feature 183..202: note = n is a, c, g or u
accgcttcaccaaaagctgtcccttaggggattagaacttgagtgaaggtgggctgcttgcatcagcctaatgtcgagaagtgctttcttcggaaagtaaccctcgaaacaaattcagtgctcctctccaattctgcacaagaaagttgcagaacccgaatagagcaatgaaggaatgcaacnnnnnnnnnnnnnnnnnnnn

SEQ ID NO: 321 - RNA, 209 nt, synthetic construct
  source 1..209: mol_type = other RNA; note = Engineered sgRNA with modification of MS1/MS4*-1
  misc_feature 190..209: note = n is a, c, g or u
cttcactgataaagtggagaaccgcttcaccaaaagctgtcccttaggggattagaacttgagtgaaggtgggctgcttgcatcagcctaatgtcgagaagtgctttcttcggaaagtaaccctcgaaacaaattcagtgctcctctccaattcgaaagaacccgaatagagcaatgaaggaatgcaacnnnnnnnnnnnnnnnnnnnn

SEQ ID NO: 322 - RNA, 197 nt, synthetic construct
  source 1..197: mol_type = other RNA; note = Engineered sgRNA with modification of MS1/MS4*-2
  misc_feature 178..197: note = n is a, c, g or u
cttcactgataaagtggagaaccgcttcaccaaaagctgtcccttaggggattagaacttgagtgaaggtgggctgcttgcatcagcctaatgtcgagaagtgctttcttcggaaagtaaccctcgaaacaaattcagtgctcctctcgaaagaatagagcaatgaaggaatgcaacnnnnnnnnnnnnnnnnnnnn

SEQ ID NO: 323 - RNA, 185 nt, synthetic construct
  source 1..185: mol_type = other RNA; note = Engineered sgRNA with modification of MS1/MS4*-3
  misc_feature 166..185: note = n is a, c, g or u
cttcactgataaagtggagaaccgcttcaccaaaagctgtcccttaggggattagaacttgagtgaaggtgggctgcttgcatcagcctaatgtcgagaagtgctttcttcggaaagtaaccctcgaaacaaattcagtgctgaaaagcaatgaaggaatgcaacnnnnnnnnnnnnnnnnnnnn

SEQ ID NO: 324 - RNA, 216 nt, synthetic construct
  source 1..216: mol_type = other RNA; note = Engineered sgRNA with modification of MS1/MS5-1
  misc_feature 197..216: note = n is a, c, g or u
cttcactgataaagtggagaaccgcttcaccaaaagctgtttagattagaacttgagtgaaggtgggctgcttgcatcagcctaatgtcgagaagtgctttcttcggaaagtaaccctcgaaacaaattcagtgctcctctccaattctgcacaagaaagttgcagaacccgaatagagcaatgaaggaatgcaacnnnnnnnnnnnnnnnnnnnn

SEQ ID NO: 325 - RNA, 209 nt, synthetic construct
  source 1..209: mol_type = other RNA; note = Engineered sgRNA with modification of MS1/MS5-2
  misc_feature 190..209: note = n is a, c, g or u
cttcactgataaagtggagaaccgcttcaccaaaagcttaggaacttgagtgaaggtgggctgcttgcatcagcctaatgtcgagaagtgctttcttcggaaagtaaccctcgaaacaaattcagtgctcctctccaattctgcacaagaaagttgcagaacccgaatagagcaatgaaggaatgcaacnnnnnnnnnnnnnnnnnnnn

SEQ ID NO: 326 - RNA, 201 nt, synthetic construct
  source 1..201: mol_type = other RNA; note = Engineered sgRNA with modification of MS1/MS5-3
  misc_feature 182..201: note = n is a, c, g or u
cttcactgataaagtggagaaccgcttcaccaattagttgagtgaaggtgggctgcttgcatcagcctaatgtcgagaagtgctttcttcggaaagtaaccctcgaaacaaattcagtgctcctctccaattctgcacaagaaagttgcagaacccgaatagagcaatgaaggaatgcaacnnnnnnnnnnnnnnnnnnnn

SEQ ID NO: 327 - RNA, 206 nt, synthetic construct
  source 1..206: mol_type = other RNA; note = Engineered sgRNA with modification of MS1/MS2/MS4*-2
  misc_feature 178..197: note = n is a, c, g or u
cttcactgataaagtggagaaccgcttcaccaaaagctgtcccttaggggattagaacttgagtgaaggtgggctgcttgcatcagcctaatgtcgagaagtgctttcttcggaaagtaaccctcgaaacaaattcagtgctcctctcgaaagaatagagcaatgaaggaatgcaacnnnnnnnnnnnnnnnnnnnnttttatttt

SEQ ID NO: 328 - RNA, 177 nt, synthetic construct
  source 1..177: mol_type = other RNA; note = Engineered sgRNA with modification of MS1/MS3-3/MS4*-2
  misc_feature 158..177: note = n is a, c, g or u
accgcttcaccaaaagctgtcccttaggggattagaacttgagtgaaggtgggctgcttgcatcagcctaatgtcgagaagtgctttcttcggaaagtaaccctcgaaacaaattcagtgctcctctcgaaagaatagagcaatgaaggaatgcaacnnnnnnnnnnnnnnnnnnnn

SEQ ID NO: 329 - RNA, 210 nt, synthetic construct
  source 1..210: mol_type = other RNA; note = Engineered sgRNA with modification of MS1/MS2/MS5-3
  misc_feature 182..201: note = n is a, c, g or u
cttcactgataaagtggagaaccgcttcaccaattagttgagtgaaggtgggctgcttgcatcagcctaatgtcgagaagtgctttcttcggaaagtaaccctcgaaacaaattcagtgctcctctccaattctgcacaagaaagttgcagaacccgaatagagcaatgaaggaatgcaacnnnnnnnnnnnnnnnnnnnnttttatttt

SEQ ID NO: 330 - RNA, 181 nt, synthetic construct
  source 1..181: mol_type = other RNA; note = Engineered sgRNA with modification of MS1/MS3-3/MS5-3
  misc_feature 162..181: note = n is a, c, g or u
accgcttcaccaattagttgagtgaaggtgggctgcttgcatcagcctaatgtcgagaagtgctttcttcggaaagtaaccctcgaaacaaattcagtgctcctctccaattctgcacaagaaagttgcagaacccgaatagagcaatgaaggaatgcaacnnnnnnnnnnnnnnnnnnnn

SEQ ID NO: 331 - RNA, 176 nt, synthetic construct
  source 1..176: mol_type = other RNA; note = Engineered sgRNA with modification of MS1/MS4*-2/MS5-3
  misc_feature 157..176: note = n is a, c, g or u
cttcactgataaagtggagaaccgcttcaccaattagttgagtgaaggtgggctgcttgcatcagcctaatgtcgagaagtgctttcttcggaaagtaaccctcgaaacaaattcagtgctcctctcgaaagaatagagcaatgaaggaatgcaacnnnnnnnnnnnnnnnnnnnn

SEQ ID NO: 332 - RNA, 186 nt, synthetic construct
  source 1..186: mol_type = other RNA; note = Engineered sgRNA with modification of MS1/MS2/MS3-3/MS4*-2
  misc_feature 158..177: note = n is a, c, g or u
accgcttcaccaaaagctgtcccttaggggattagaacttgagtgaaggtgggctgcttgcatcagcctaatgtcgagaagtgctttcttcggaaagtaaccctcgaaacaaattcagtgctcctctcgaaagaatagagcaatgaaggaatgcaacnnnnnnnnnnnnnnnnnnnnttttatttt

SEQ ID NO: 333 - RNA, 190 nt, synthetic construct
  source 1..190: mol_type = other RNA; note = Engineered sgRNA with modification of MS1/MS2/MS3-3/MS5-3
  misc_feature 162..181: note = n is a, c, g or u
accgcttcaccaattagttgagtgaaggtgggctgcttgcatcagcctaatgtcgagaagtgctttcttcggaaagtaaccctcgaaacaaattcagtgctcctctccaattctgcacaagaaagttgcagaacccgaatagagcaatgaaggaatgcaacnnnnnnnnnnnnnnnnnnnnttttatttt

SEQ ID NO: 334 - RNA, 185 nt, synthetic construct
  source 1..185: mol_type = other RNA; note = Engineered sgRNA with modification of MS1/MS2/MS4*-2/MS5-3
  misc_feature 157..176: note = n is a, c, g or u
cttcactgataaagtggagaaccgcttcaccaattagttgagtgaaggtgggctgcttgcatcagcctaatgtcgagaagtgctttcttcggaaagtaaccctcgaaacaaattcagtgctcctctcgaaagaatagagcaatgaaggaatgcaacnnnnnnnnnnnnnnnnnnnnttttatttt

SEQ ID NO: 335 - RNA, 156 nt, synthetic construct
  source 1..156: mol_type = other RNA; note = Engineered sgRNA with modification of MS1/MS3-3/MS4*-2/MS5-3
  misc_feature 137..156: note = n is a, c, g or u
accgcttcaccaattagttgagtgaaggtgggctgcttgcatcagcctaatgtcgagaagtgctttcttcggaaagtaaccctcgaaacaaattcagtgctcctctcgaaagaatagagcaatgaaggaatgcaacnnnnnnnnnnnnnnnnnnnn

SEQ ID NO: 336 - RNA, 165 nt, synthetic construct
  source 1..165: mol_type = other RNA; note = Engineered sgRNA with modification of MS1/MS2/MS3-3/MS4*-2/MS5-3
  misc_feature 137..156: note = n is a, c, g or u
accgcttcaccaattagttgagtgaaggtgggctgcttgcatcagcctaatgtcgagaagtgctttcttcggaaagtaaccctcgaaacaaattcagtgctcctctcgaaagaatagagcaatgaaggaatgcaacnnnnnnnnnnnnnnnnnnnnttttatttt

SEQ ID NO: 337 - RNA, 181 nt, synthetic construct
  source 1..181: mol_type = other RNA; note = Mature form sgRNA
  misc_feature 162..181: note = n is a, c, g or u
cttcactgataaagtggagaaccgcttcaccaaaagctgtcccttaggggattagaacttgagtgaaggtgggctgcttgcatcagcctaatgtcgagaagtgctttcttcggaaagtaaccctcgaaacaaattcatttgaaagaatgaaggaatgcaacnnnnnnnnnnnnnnnnnnnn

SEQ ID NO: 338 - RNA, 174 nt, synthetic construct
  source 1..174: mol_type = other RNA; note = Mature form sgRNA with modification of MS3-1
  misc_feature 155..174: note = n is a, c, g or u
gataaagtggagaaccgcttcaccaaaagctgtcccttaggggattagaacttgagtgaaggtgggctgcttgcatcagcctaatgtcgagaagtgctttcttcggaaagtaaccctcgaaacaaattcatttgaaagaatgaaggaatgcaacnnnnnnnnnnnnnnnnnnnn

SEQ ID NO: 339 - RNA, 167 nt, synthetic construct
  source 1..167: mol_type = other RNA; note = Mature form sgRNA with modification of MS3-2
  misc_feature 148..167: note = n is a, c, g or u
tggagaaccgcttcaccaaaagctgtcccttaggggattagaacttgagtgaaggtgggctgcttgcatcagcctaatgtcgagaagtgctttcttcggaaagtaaccctcgaaacaaattcatttgaaagaatgaaggaatgcaacnnnnnnnnnnnnnnnnnnnn

SEQ ID NO: 340 - RNA, 161 nt, synthetic construct
  source 1..161: mol_type = other RNA; note = Mature form sgRNA with modification of MS3-3
  misc_feature 142..161: note = n is a, c, g or u
accgcttcaccaaaagctgtcccttaggggattagaacttgagtgaaggtgggctgcttgcatcagcctaatgtcgagaagtgctttcttcggaaagtaaccctcgaaacaaattcatttgaaagaatgaaggaatgcaacnnnnnnnnnnnnnnnnnnnn

SEQ ID NO: 341 - RNA, 177 nt, synthetic construct
  source 1..177: mol_type = other RNA; note = Mature form sgRNA with modification of MS4-1
  misc_feature 158..177: note = n is a, c, g or u
cttcactgataaagtggagaaccgcttcaccaaaagctgtcccttaggggattagaacttgagtgaaggtgggctgcttgcatcagcctaatgtcgagaagtgctttcttcggaaagtaaccctcgaaacaaattcatgaaaatgaaggaatgcaacnnnnnnnnnnnnnnnnnnnn

SEQ ID NO: 342 - RNA, 173 nt, synthetic construct
  source 1..173: mol_type = other RNA; note = Mature form sgRNA with modification of MS4-2
  misc_feature 154..173: note = n is a, c, g or u
cttcactgataaagtggagaaccgcttcaccaaaagctgtcccttaggggattagaacttgagtgaaggtgggctgcttgcatcagcctaatgtcgagaagtgctttcttcggaaagtaaccctcgaaacaaattcgaaagaaggaatgcaacnnnnnnnnnnnnnnnnnnnn

SEQ ID NO: 343 - RNA, 167 nt, synthetic construct
  source 1..167: mol_type = other RNA; note = Mature form sgRNA with modification of MS4-3
  misc_feature 148..167: note = n is a, c, g or u
cttcactgataaagtggagaaccgcttcaccaaaagctgtcccttaggggattagaacttgagtgaaggtgggctgcttgcatcagcctaatgtcgagaagtgctttcttcggaaagtaaccctcgaaacaaagaaaggaatgcaacnnnnnnnnnnnnnnnnnnnn

SEQ ID NO: 344 - RNA, 175 nt, synthetic construct
  source 1..175: mol_type = other RNA; note = Mature form sgRNA with modification of MS5-1
  misc_feature 156..175: note = n is a, c, g or u
cttcactgataaagtggagaaccgcttcaccaaaagctgtttagattagaacttgagtgaaggtgggctgcttgcatcagcctaatgtcgagaagtgctttcttcggaaagtaaccctcgaaacaaattcatttgaaagaatgaaggaatgcaacnnnnnnnnnnnnnnnnnnnn

SEQ ID NO: 345 - RNA, 170 nt, synthetic construct
  source 1..170: mol_type = other RNA; note = Mature form sgRNA with modification of MS5-2
  misc_feature 151..170: note = n is a, c, g or u
cttcactgataaagtggagaaccgcttcaccaaaagctttagagaacttgagtgaaggtgggctgcttgcatcagcctaatgtcgagaagtgctttcttcggaaagtaaccctcgaaacaaattcatttgaaagaatgaaggaatgcaacnnnnnnnnnnnnnnnnnnnn

SEQ ID NO: 346 - RNA, 160 nt, synthetic construct
  source 1..160: mol_type = other RNA; note = Mature form sgRNA with modification of MS5-3
  misc_feature 141..160: note = n is a, c, g or u
cttcactgataaagtggagaaccgcttcaccaattagttgagtgaaggtgggctgcttgcatcagcctaatgtcgagaagtgctttcttcggaaagtaaccctcgaaacaaattcatttgaaagaatgaaggaatgcaacnnnnnnnnnnnnnnnnnnnn

SEQ ID NO: 347 - RNA, 147 nt, synthetic construct
  source 1..147: mol_type = other RNA; note = Mature form sgRNA with modification of MS3-3/MS4-3
  misc_feature 128..147: note = n is a, c, g or u
accgcttcaccaaaagctgtcccttaggggattagaacttgagtgaaggtgggctgcttgcatcagcctaatgtcgagaagtgctttcttcggaaagtaaccctcgaaacaaagaaaggaatgcaacnnnnnnnnnnnnnnnnnnnn

SEQ ID NO: 348 - RNA, 140 nt, synthetic construct
  source 1..140: mol_type = other RNA; note = Mature form sgRNA with modification of MS3-3/MS5-3
  misc_feature 121..140: note = n is a, c, g or u
accgcttcaccaattagttgagtgaaggtgggctgcttgcatcagcctaatgtcgagaagtgctttcttcggaaagtaaccctcgaaacaaattcatttgaaagaatgaaggaatgcaacnnnnnnnnnnnnnnnnnnnn

SEQ ID NO: 349 - RNA, 146 nt, synthetic construct
  source 1..146: mol_type = other RNA; note = Mature form sgRNA with modification of MS4-3/MS5-3
  misc_feature 127..146: note = n is a, c, g or u
cttcactgataaagtggagaaccgcttcaccaattagttgagtgaaggtgggctgcttgcatcagcctaatgtcgagaagtgctttcttcggaaagtaaccctcgaaacaaagaaaggaatgcaacnnnnnnnnnnnnnnnnnnnn

SEQ ID NO: 350 - RNA, 126 nt, synthetic construct
  source 1..126: mol_type = other RNA; note = Mature form sgRNA with modification of MS3-3/MS4-3/MS5-3
  misc_feature 107..126: note = n is a, c, g or u
accgcttcaccaattagttgagtgaaggtgggctgcttgcatcagcctaatgtcgagaagtgctttcttcggaaagtaaccctcgaaacaaagaaaggaatgcaacnnnnnnnnnnnnnnnnnnnn

SEQ ID NO: 351 - RNA, 10 nt, synthetic construct
  source 1..10: mol_type = other RNA; note = U-rich tail
tttttttttt

SEQ ID NO: 352 - RNA, 10 nt, synthetic construct
  source 1..10: mol_type = other RNA; note = U-rich tail
ttatttattt

SEQ ID NO: 353 - RNA, 10 nt, synthetic construct
  source 1..10: mol_type = other RNA; note = U-rich tail
tttctatttt

SEQ ID NO: 354 - RNA, 10 nt, synthetic construct
  source 1..10: mol_type = other RNA; note = U-rich tail
ttatgttttt

SEQ ID NO: 355 - RNA, 10 nt, synthetic construct
  source 1..10: mol_type = other RNA; note = The additional sequence for engineered Cas protein gRNA
ataaaggtga

SEQ ID NO: 356 - RNA, 37 nt, synthetic construct
  source 1..37: mol_type = other RNA; note = The additional sequence for engineered Cas protein gRNA
ctgatgagtccgtgaggacgaaacgagtaagctcgtc

SEQ ID NO: 357 - RNA, 37 nt, synthetic construct
  source 1..37: mol_type = other RNA; note = The additional sequence for engineered Cas protein gRNA
ctgctcgaatgagcaaagcaggagtgcctgagtagtc

SEQ ID NO: 358 - DNA, 24 bp, synthetic construct
  source 1..24: mol_type = other DNA; note = Target-1 sequence
tttgcacacacacagtgggctacc

SEQ ID NO: 359 - DNA, 24 bp, synthetic construct
  source 1..24: mol_type = other DNA; note = Target-2 sequence
tttgcatccccaggacacacacac

SEQ ID NO: 360 - protein, 557 aa, unidentified
  source 1..557: note = CWCas12f1
MGEKSSRRRRNGKSGAWTAAITSCVGGKMAKNTITKTLKLRIVRPYNSAEVEKIVADEKNNREKIALEKNKDKVKEACSKHLKVAAYCTTQVERNACLFCKARKLDDKFYQKLRGQFPDAVFWQEISEIFRQLQKQAAEIYNQSLIELYYEIFIKGKGIANASSVEHYLSDVCYTRAAELFKNAAIASGLRSKIKSNFRLKELKNMKSGLPTTKSDNFPIPLVKQKGGQYTGFEISNHNSDFIIKIPFGRWQVKKEIDKYRPWEKFDFEQVQKSPKPISLLLSTQRRKRNKGWSKDEGTEAEIKKVMNGDYQTSYIEVKRGSKIGEKSAWMLNLSIDVPKIDKGVDPSIIGGIDVGVKSPLVCAINNAFSRYSISDNDLFHFNKKMFARRRILLKKNRHKRAGHGAKNKLKPITILTEKSERFRKKLIERWACEIADFFIKNKVGTVQMENLESMKRKEDSYFNIRLRGFWPYAEMQNKIEFKLKQYGIEIRKVAPNNTSKTCSKCGHLNNYFNFEYRKKNKFPHFKCEKCNFKENADYNAALNISNPKLKSTKEEP

SEQ ID NO: 361 - protein, 555 aa, synthetic construct
  source 1..555: note = CWCas12f1 variant 1
MEKRINKIRKKLSADNATKPVSRSGPMAKNTITKTLKLRIVRPYNSAEVEKIVADEKNNREKIALEKNKDKVKEACSKHLKVAAYCTTQVERNACLFCKARKLDDKFYQKLRGQFPDAVFWQEISEIFRQLQKQAAEIYNQSLIELYYEIFIKGKGIANASSVEHYLSDVCYTRAAELFKNAAIASGLRSKIKSNFRLKELKNMKSGLPTTKSDNFPIPLVKQKGGQYTGFEISNHNSDFIIKIPFGRWQVKKEIDKYRPWEKFDFEQVQKSPKPISLLLSTQRRKRNKGWSKDEGTEAEIKKVMNGDYQTSYIEVKRGSKIGEKSAWMLNLSIDVPKIDKGVDPSIIGGIDVGVKSPLVCAINNAFSRYSISDNDLFHFNKKMFARRRILLKKNRHKRAGHGAKNKLKPITILTEKSERFRKKLIERWACEIADFFIKNKVGTVQMENLESMKRKEDSYFNIRLRGFWPYAEMQNKIEFKLKQYGIEIRKVAPNNTSKTCSKCGHLNNYFNFEYRKKNKFPHFKCEKCNFKENADYNAALNISNPKLKSTKEEP

SEQ ID NO: 362 - protein, 557 aa, synthetic construct
  source 1..557: note = CWCas12f1 variant 2
MAGGPGAGSAAPVSSTSSLPLAALNMRVMAKNTITKTLKLRIVRPYNSAEVEKIVADEKNNREKIALEKNKDKVKEACSKHLKVAAYCTTQVERNACLFCKARKLDDKFYQKLRGQFPDAVFWQEISEIFRQLQKQAAEIYNQSLIELYYEIFIKGKGIANASSVEHYLSDVCYTRAAELFKNAAIASGLRSKIKSNFRLKELKNMKSGLPTTKSDNFPIPLVKQKGGQYTGFEISNHNSDFIIKIPFGRWQVKKEIDKYRPWEKFDFEQVQKSPKPISLLLSTQRRKRNKGWSKDEGTEAEIKKVMNGDYQTSYIEVKRGSKIGEKSAWMLNLSIDVPKIDKGVDPSIIGGIDVGVKSPLVCAINNAFSRYSISDNDLFHFNKKMFARRRILLKKNRHKRAGHGAKNKLKPITILTEKSERFRKKLIERWACEIADFFIKNKVGTVQMENLESMKRKEDSYFNIRLRGFWPYAEMQNKIEFKLKQYGIEIRKVAPNNTSKTCSKCGHLNNYFNFEYRKKNKFPHFKCEKCNFKENADYNAALNISNPKLKSTKEEP

SEQ ID NO: 363 - protein, 555 aa, synthetic construct
  source 1..555: note = CWCas12f1 variant 3
MAGGPGAGSAAPVSSTSSLPLAALNMMAKNTITKTLKLRIVRPYNSAEVEKIVADEKNNREKIALEKNKDKVKEACSKHLKVAAYCTTQVERNACLFCKARKLDDKFYQKLRGQFPDAVFWQEISEIFRQLQKQAAEIYNQSLIELYYEIFIKGKGIANASSVEHYLSDVCYTRAAELFKNAAIASGLRSKIKSNFRLKELKNMKSGLPTTKSDNFPIPLVKQKGGQYTGFEISNHNSDFIIKIPFGRWQVKKEIDKYRPWEKFDFEQVQKSPKPISLLLSTQRRKRNKGWSKDEGTEAEIKKVMNGDYQTSYIEVKRGSKIGEKSAWMLNLSIDVPKIDKGVDPSIIGGIDVGVKSPLVCAINNAFSRYSISDNDLFHFNKKMFARRRILLKKNRHKRAGHGAKNKLKPITILTEKSERFRKKLIERWACEIADFFIKNKVGTVQMENLESMKRKEDSYFNIRLRGFWPYAEMQNKIEFKLKQYGIEIRKVAPNNTSKTCSKCGHLNNYFNFEYRKKNKFPHFKCEKCNFKENADYNAALNISNPKLKSTKEEP

SEQ ID NO: 364 - protein, 529 aa, unidentified
  source 1..529: note = Un1Cas12f1
MAKNTITKTLKLRIVRPYNSAEVEKIVADEKNNREKIALEKNKDKVKEACSKHLKVAAYCTTQVERNACLFCKARKLDDKFYQKLRGQFPDAVFWQEISEIFRQLQKQAAEIYNQSLIELYYEIFIKGKGIANASSVEHYLSDVCYTRAAELFKNAAIASGLRSKIKSNFRLKELKNMKSGLPTTKSDNFPIPLVKQKGGQYTGFEISNHNSDFIIKIPFGRWQVKKEIDKYRPWEKFDFEQVQKSPKPISLLLSTQRRKRNKGWSKDEGTEAEIKKVMNGDYQTSYIEVKRGSKIGEKSAWMLNLSIDVPKIDKGVDPSIIGGIDVGVKSPLVCAINNAFSRYSISDNDLFHFNKKMFARRRILLKKNRHKRAGHGAKNKLKPITILTEKSERFRKKLIERWACEIADFFIKNKVGTVQMENLESMKRKEDSYFNIRLRGFWPYAEMQNKIEFKLKQYGIEIRKVAPNNTSKTCSKCGHLNNYFNFEYRKKNKFPHFKCEKCNFKENADYNAALNISNPKLKSTKEEP

SEQ ID NO: 365 - DNA, 1671 bp, synthetic construct
  source 1..1671: mol_type = other DNA; note = Human codon-optimized CWCas12f1
atgggggagaaaagttcccgccgccgacggaatggaaaaagcggtgcgtggactgctgctataacaagctgtgttgggggtaagatggccaagaacacaattacaaagacactgaagctgaggatcgtgagaccatacaacagcgctgaggtcgagaagattgtggctgatgaaaagaacaacagggaaaagatcgccctcgagaagaacaaggataaggtgaaggaggcctgctctaagcacctgaaagtggccgcctactgcaccacacaggtggagaggaacgcctgtctgttttgtaaagctcggaagctggatgataagttttaccagaagctgcggggccagttccccgatgccgtcttttggcaggagattagcgagatcttcagacagctgcagaagcaggccgccgagatctacaaccagagcctgatcgagctctactacgagatcttcatcaagggcaagggcattgccaacgcctcctccgtggagcactacctgagcgacgtgtgctacacaagagccgccgagctctttaagaacgccgctatcgcttccgggctgaggagcaagattaagagtaacttccggctcaaggagctgaagaacatgaagagcggcctgcccactacaaagagcgacaacttcccaattccactggtgaagcagaaggggggccagtacacagggttcgagatttccaaccacaacagcgactttattattaagatcccctttggcaggtggcaggtcaagaaggagattgacaagtacaggccctgggagaagtttgatttcgagcaggtgcagaagagccccaagcctatttccctgctgctgtccacacagcggcggaagaggaacaaggggtggtctaaggatgaggggaccgaggccgagattaagaaagtgatgaacggcgactaccagacaagctacatcgaggtcaagcggggcagtaagattggcgagaagagcgcctggatgctgaacctgagcattgacgtgccaaagattgataagggcgtggatcccagcatcatcggagggatcgatgtgggggtcaagagccccctcgtgtgcgccatcaacaacgccttcagcaggtacagcatctccgataacgacctgttccactttaacaagaagatgttcgcccggcggaggattttgctcaagaagaaccggcacaagcgggccggacacggggccaagaacaagctcaagcccatcactatcctgaccgagaagagcgagaggttcaggaagaagctcatcgagagatgggcctgcgagatcgccgatttctttattaagaacaaggtcggaacagtgcagatggagaacctcgagagcatgaagaggaaggaggattcctacttcaacattcggctgagggggttctggccctacgctgagatgcagaacaagattgagtttaagctgaagcagtacgggattgagatccggaaggtggcccccaacaacaccagcaagacctgcagcaagtgcgggcacctcaacaactacttcaacttcgagtaccggaagaagaacaagttcccacacttcaagtgcgagaagtgcaactttaaggagaacgccgattacaacgccgccctgaacatcagcaaccctaagctgaagagcactaaggaggagccc

SEQ ID NO: 366 - DNA, 1666 bp, synthetic construct
  source 1..1666: mol_type = other DNA; note = Human codon-optimized CWCas12f1 variant 1
atggaaaagagaatcaacaagatcaggaagaagctgagcgccgacaacgccaccaagcctgtgtctaggagtggcccccatggccaagaacacaattacaaagacactgaagctgaggatcgtgagaccatacaacagcgctgaggtcgagaagattgtggctgatgaaaagaacaacagggaaaagatcgccctcgagaagaacaaggataaggtgaaggaggcctgctctaagcacctgaaagtggccgcctactgcaccacacaggtggagaggaacgcctgtctgttttgtaaagctcggaagctggatgataagttttaccagaagctgcggggccagttccccgatgccgtcttttggcaggagattagcgagatcttcagacagctgcagaagcaggccgccgagatctacaaccagagcctgatcgagctctactacgagatcttcatcaagggcaagggcattgccaacgcctcctccgtggagcactacctgagcgacgtgtgctacacaagagccgccgagctctttaagaacgccgctatcgcttccgggctgaggagcaagattaagagtaacttccggctcaaggagctgaagaacatgaagagcggcctgcccactacaaagagcgacaacttcccaattccactggtgaagcagaaggggggccagtacacagggttcgagatttccaaccacaacagcgactttattattaagatcccctttggcaggtggcaggtcaagaaggagattgacaagtacaggccctgggagaagtttgatttcgagcaggtgcagaagagccccaagcctatttccctgctgctgtccacacagcggcggaagaggaacaaggggtggtctaaggatgaggggaccgaggccgagattaagaaagtgatgaacggcgactaccagacaagctacatcgaggtcaagcggggcagtaagattggcgagaagagcgcctggatgctgaacctgagcattgacgtgccaaagattgataagggcgtggatcccagcatcatcggagggatcgatgtgggggtcaagagccccctcgtgtgcgccatcaacaacgccttcagcaggtacagcatctccgataacgacctgttccactttaacaagaagatgttcgcccggcggaggattttgctcaagaagaaccggcacaagcgggccggacacggggccaagaacaagctcaagcccatcactatcctgaccgagaagagcgagaggttcaggaagaagctcatcgagagatgggcctgcgagatcgccgatttctttattaagaacaaggtcggaacagtgcagatggagaacctcgagagcatgaagaggaaggaggattcctacttcaacattcggctgagggggttctggccctacgctgagatgcagaacaagattgagtttaagctgaagcagtacgggattgagatccggaaggtggcccccaacaacaccagcaagacctgcagcaagtgcgggcacctcaacaactacttcaacttcgagtaccggaagaagaacaagttcccacacttcaagtgcgagaagtgcaactttaaggagaacgccgattacaacgccgccctgaacatcagcaaccctaagctgaagagcactaaggaggagccc

SEQ ID NO: 367 - DNA, 1671 bp, synthetic construct
  source 1..1671: mol_type = other DNA; note = Human codon-optimized CWCas12f1 variant 2
atggctggcggaccaggcgcaggtagtgctgcgccagtttcttcaacttcctccctgcccctggctgcgcttaacatgcgcgtgatggccaagaacacaattacaaagacactgaagctgaggatcgtgagaccatacaacagcgctgaggtcgagaagattgtggctgatgaaaagaacaacagggaaaagatcgccctcgagaagaacaaggataaggtgaaggaggcctgctctaagcacctgaaagtggccgcctactgcaccacacaggtggagaggaacgcctgtctgttttgtaaagctcggaagctggatgataagttttaccagaagctgcggggccagttccccgatgccgtcttttggcaggagattagcgagatcttcagacagctgcagaagcaggccgccgagatctacaaccagagcctgatcgagctctactacgagatcttcatcaagggcaagggcattgccaacgcctcctccgtggagcactacctgagcgacgtgtgctacacaagagccgccgagctctttaagaacgccgctatcgcttccgggctgaggagcaagattaagagtaacttccggctcaaggagctgaagaacatgaagagcggcctgcccactacaaagagcgacaacttcccaattccactggtgaagcagaaggggggccagtacacagggttcgagatttccaaccacaacagcgactttattattaagatcccctttggcaggtggcaggtcaagaaggagattgacaagtacaggccctgggagaagtttgatttcgagcaggtgcagaagagccccaagcctatttccctgctgctgtccacacagcggcggaagaggaacaaggggtggtctaaggatgaggggaccgaggccgagattaagaaagtgatgaacggcgactaccagacaagctacatcgaggtcaagcggggcagtaagattggcgagaagagcgcctggatgctgaacctgagcattgacgtgccaaagattgataagggcgtggatcccagcatcatcggagggatcgatgtgggggtcaagagccccctcgtgtgcgccatcaacaacgccttcagcaggtacagcatctccgataacgacctgttccactttaacaagaagatgttcgcccggcggaggattttgctcaagaagaaccggcacaagcgggccggacacggggccaagaacaagctcaagcccatcactatcctgaccgagaagagcgagaggttcaggaagaagctcatcgagagatgggcctgcgagatcgccgatttctttattaagaacaaggtcggaacagtgcagatggagaacctcgagagcatgaagaggaaggaggattcctacttcaacattcggctgagggggttctggccctacgctgagatgcagaacaagattgagtttaagctgaagcagtacgggattgagatccggaaggtggcccccaacaacaccagcaagacctgcagcaagtgcgggcacctcaacaactacttcaacttcgagtaccggaagaagaacaagttcccacacttcaagtgcgagaagtgcaactttaaggagaacgccgattacaacgccgccctgaacatcagcaaccctaagctgaagagcactaaggaggagccc

SEQ ID NO: 368 - DNA, 1665 bp, synthetic construct
  source 1..1665: mol_type = other DNA; note = Human codon-optimized CWCas12f1 variant 3
atggctggcggaccaggcgcaggtagtgctgcgccagtttcttcaacttcctccctgcccctggctgcgcttaacatgatggccaagaacacaattacaaagacactgaagctgaggatcgtgagaccatacaacagcgctgaggtcgagaagattgtggctgatgaaaagaacaacagggaaaagatcgccctcgagaagaacaaggataaggtgaaggaggcctgctctaagcacctgaaagtggccgcctactgcaccacacaggtggagaggaacgcctgtctgttttgtaaagctcggaagctggatgataagttttaccagaagctgcggggccagttccccgatgccgtcttttggcaggagattagcgagatcttcagacagctgcagaagcaggccgccgagatctacaaccagagcctgatcgagctctactacgagatcttcatcaagggcaagggcattgccaacgcctcctccgtggagcactacctgagcgacgtgtgctacacaagagccgccgagctctttaagaacgccgctatcgcttccgggctgaggagcaagattaagagtaacttccggctcaaggagctgaagaacatgaagagcggcctgcccactacaaagagcgacaacttcccaattccactggtgaagcagaaggggggccagtacacagggttcgagatttccaaccacaacagcgactttattattaagatcccctttggcaggtggcaggtcaagaaggagattgacaagtacaggccctgggagaagtttgatttcgagcaggtgcagaagagccccaagcctatttccctgctgctgtccacacagcggcggaagaggaacaaggggtggtctaaggatgaggggaccgaggccgagattaagaaagtgatgaacggcgactaccagacaagctacatcgaggtcaagcggggcagtaagattggcgagaagagcgcctggatgctgaacctgagcattgacgtgccaaagattgataagggcgtggatcccagcatcatcggagggatcgatgtgggggtcaagagccccctcgtgtgcgccatcaacaacgccttcagcaggtacagcatctccgataacgacctgttccactttaacaagaagatgttcgcccggcggaggattttgctcaagaagaaccggcacaagcgggccggacacggggccaagaacaagctcaagcccatcactatcctgaccgagaagagcgagaggttcaggaagaagctcatcgagagatgggcctgcgagatcgccgatttctttattaagaacaaggtcggaacagtgcagatggagaacctcgagagcatgaagaggaaggaggattcctacttcaacattcggctgagggggttctggccctacgctgagatgcagaacaagattgagtttaagctgaagcagtacgggattgagatccggaaggtggcccccaacaacaccagcaagacctgcagcaagtgcgggcacctcaacaactacttcaacttcgagtaccggaagaagaacaagttcccacacttcaagtgcgagaagtgcaactttaaggagaacgccgattacaacgccgccctgaacatcagcaaccctaagctgaagagcactaaggaggagccc

SEQ ID NO: 369 - DNA, 1587 bp, synthetic construct
  source 1..1587: mol_type = other DNA; note = Human codon-optimized Un1Cas12f1
atggccaagaacacaattacaaagacactgaagctgaggatcgtgagaccatacaacagcgctgaggtcgagaagattgtggctgatgaaaagaacaacagggaaaagatcgccctcgagaagaacaaggataaggtgaaggaggcctgctctaagcacctgaaagtggccgcctactgcaccacacaggtggagaggaacgcctgtctgttttgtaaagctcggaagctggatgataagttttaccagaagctgcggggccagttccccgatgccgtcttttggcaggagattagcgagatcttcagacagctgcagaagcaggccgccgagatctacaaccagagcctgatcgagctctactacgagatcttcatcaagggcaagggcattgccaacgcctcctccgtggagcactacctgagcgacgtgtgctacacaagagccgccgagctctttaagaacgccgctatcgcttccgggctgaggagcaagattaagagtaacttccggctcaaggagctgaagaacatgaagagcggcctgcccactacaaagagcgacaacttcccaattccactggtgaagcagaaggggggccagtacacagggttcgagatttccaaccacaacagcgactttattattaagatcccctttggcaggtggcaggtcaagaaggagattgacaagtacaggccctgggagaagtttgatttcgagcaggtgcagaagagccccaagcctatttccctgctgctgtccacacagcggcggaagaggaacaaggggtggtctaaggatgaggggaccgaggccgagattaagaaagtgatgaacggcgactaccagacaagctacatcgaggtcaagcggggcagtaagattggcgagaagagcgcctggatgctgaacctgagcattgacgtgccaaagattgataagggcgtggatcccagcatcatcggagggatcgatgtgggggtcaagagccccctcgtgtgcgccatcaacaacgccttcagcaggtacagcatctccgataacgacctgttccactttaacaagaagatgttcgcccggcggaggattttgctcaagaagaaccggcacaagcgggccggacacggggccaagaacaagctcaagcccatcactatcctgaccgagaagagcgagaggttcaggaagaagctcatcgagagatgggcctgcgagatcgccgatttctttattaagaacaaggtcggaacagtgcagatggagaacctcgagagcatgaagaggaaggaggattcctacttcaacattcggctgagggggttctggccctacgctgagatgcagaacaagattgagtttaagctgaagcagtacgggattgagatccggaaggtggcccccaacaacaccagcaagacctgcagcaagtgcgggcacctcaacaactacttcaacttcgagtaccggaagaagaacaagttcccacacttcaagtgcgagaagtgcaactttaaggagaacgccgattacaacgccgccctgaacatcagcaaccctaagctgaagagcactaaggaggagccc

SEQ ID NO: 370 - protein, 557 aa, synthetic construct
  source 1..557: note = Engineered CWCas12f1 (S170T)
MGEKSSRRRRNGKSGAWTAAITSCVGGKMAKNTITKTLKLRIVRPYNSAEVEKIVADEKNNREKIALEKNKDKVKEACSKHLKVAAYCTTQVERNACLFCKARKLDDKFYQKLRGQFPDAVFWQEISEIFRQLQKQAAEIYNQSLIELYYEIFIKGKGIANASSVEHYLTDVCYTRAAELFKNAAIASGLRSKIKSNFRLKELKNMKSGLPTTKSDNFPIPLVKQKGGQYTGFEISNHNSDFIIKIPFGRWQVKKEIDKYRPWEKFDFEQVQKSPKPISLLLSTQRRKRNKGWSKDEGTEAEIKKVMNGDYQTSYIEVKRGSKIGEKSAWMLNLSIDVPKIDKGVDPSIIGGIDVGVKSPLVCAINNAFSRYSISDNDLFHFNKKMFARRRILLKKNRHKRAGHGAKNKLKPITILTEKSERFRKKLIERWACEIADFFIKNKVGTVQMENLESMKRKEDSYFNIRLRGFWPYAEMQNKIEFKLKQYGIEIRKVAPNNTSKTCSKCGHLNNYFNFEYRKKNKFPHFKCEKCNFKENADYNAALNISNPKLKSTKEEP

SEQ ID NO: 371 - protein, 557 aa, synthetic construct
  source 1..557: note = Engineered CWCas12f1 (S188Q)
MGEKSSRRRRNGKSGAWTAAITSCVGGKMAKNTITKTLKLRIVRPYNSAEVEKIVADEKNNREKIALEKNKDKVKEACSKHLKVAAYCTTQVERNACLFCKARKLDDKFYQKLRGQFPDAVFWQEISEIFRQLQKQAAEIYNQSLIELYYEIFIKGKGIANASSVEHYLSDVCYTRAAELFKNAAIAQGLRSKIKSNFRLKELKNMKSGLPTTKSDNFPIPLVKQKGGQYTGFEISNHNSDFIIKIPFGRWQVKKEIDKYRPWEKFDFEQVQKSPKPISLLLSTQRRKRNKGWSKDEGTEAEIKKVMNGDYQTSYIEVKRGSKIGEKSAWMLNLSIDVPKIDKGVDPSIIGGIDVGVKSPLVCAINNAFSRYSISDNDLFHFNKKMFARRRILLKKNRHKRAGHGAKNKLKPITILTEKSERFRKKLIERWACEIADFFIKNKVGTVQMENLESMKRKEDSYFNIRLRGFWPYAEMQNKIEFKLKQYGIEIRKVAPNNTSKTCSKCGHLNNYFNFEYRKKNKFPHFKCEKCNFKENADYNAALNISNPKLKSTKEEP

SEQ ID NO: 372 - protein, 557 aa, synthetic construct
  source 1..557: note = Engineered CWCas12f1 (S188H)
MGEKSSRRRRNGKSGAWTAAITSCVGGKMAKNTITKTLKLRIVRPYNSAEVEKIVADEKNNREKIALEKNKDKVKEACSKHLKVAAYCTTQVERNACLFCKARKLDDKFYQKLRGQFPDAVFWQEISEIFRQLQKQAAEIYNQSLIELYYEIFIKGKGIANASSVEHYLSDVCYTRAAELFKNAAIAHGLRSKIKSNFRLKELKNMKSGLPTTKSDNFPIPLVKQKGGQYTGFEISNHNSDFIIKIPFGRWQVKKEIDKYRPWEKFDFEQVQKSPKPISLLLSTQRRKRNKGWSKDEGTEAEIKKVMNGDYQTSYIEVKRGSKIGEKSAWMLNLSIDVPKIDKGVDPSIIGGIDVGVKSPLVCAINNAFSRYSISDNDLFHFNKKMFARRRILLKKNRHKRAGHGAKNKLKPITILTEKSERFRKKLIERWACEIADFFIKNKVGTVQMENLESMKRKEDSYFNIRLRGFWPYAEMQNKIEFKLKQYGIEIRKVAPNNTSKTCSKCGHLNNYFNFEYRKKNKFPHFKCEKCNFKENADYNAALNISNPKLKSTKEEP

SEQ ID NO: 373 - protein, 557 aa, synthetic construct
  source 1..557: note = Engineered CWCas12f1 (S188K)
MGEKSSRRRRNGKSGAWTAAITSCVGGKMAKNTITKTLKLRIVRPYNSAEVEKIVADEKNNREKIALEKNKDKVKEACSKHLKVAAYCTTQVERNACLFCKARKLDDKFYQKLRGQFPDAVFWQEISEIFRQLQKQAAEIYNQSLIELYYEIFIKGKGIANASSVEHYLSDVCYTRAAELFKNAAIAKGLRSKIKSNFRLKELKNMKSGLPTTKSDNFPIPLVKQKGGQYTGFEISNHNSDFIIKIPFGRWQVKKEIDKYRPWEKFDFEQVQKSPKPISLLLSTQRRKRNKGWSKDEGTEAEIKKVMNGDYQTSYIEVKRGSKIGEKSAWMLNLSIDVPKIDKGVDPSIIGGIDVGVKSPLVCAINNAFSRYSISDNDLFHFNKKMFARRRILLKKNRHKRAGHGAKNKLKPITILTEKSERFRKKLIERWACEIADFFIKNKVGTVQMENLESMKRKEDSYFNIRLRGFWPYAEMQNKIEFKLKQYGIEIRKVAPNNTSKTCSKCGHLNNYFNFEYRKKNKFPHFKCEKCNFKENADYNAALNISNPKLKSTKEEP

SEQ ID NO: 374 - protein, 557 aa, synthetic construct
  source 1..557: note = Engineered CWCas12f1 (R191K)
MGEKSSRRRRNGKSGAWTAAITSCVGGKMAKNTITKTLKLRIVRPYNSAEVEKIVADEKNNREKIALEKNKDKVKEACSKHLKVAAYCTTQVERNACLFCKARKLDDKFYQKLRGQFPDAVFWQEISEIFRQLQKQAAEIYNQSLIELYYEIFIKGKGIANASSVEHYLSDVCYTRAAELFKNAAIASGLKSKIKSNFRLKELKNMKSGLPTTKSDNFPIPLVKQKGGQYTGFEISNHNSDFIIKIPFGRWQVKKEIDKYRPWEKFDFEQVQKSPKPISLLLSTQRRKRNKGWSKDEGTEAEIKKVMNGDYQTSYIEVKRGSKIGEKSAWMLNLSIDVPKIDKGVDPSIIGGIDVGVKSPLVCAINNAFSRYSISDNDLFHFNKKMFARRRILLKKNRHKRAGHGAKNKLKPITILTEKSERFRKKLIERWACEIADFFIKNKVGTVQMENLESMKRKEDSYFNIRLRGFWPYAEMQNKIEFKLKQYGIEIRKVAPNNTSKTCSKCGHLNNYFNFEYRKKNKFPHFKCEKCNFKENADYNAALNISNPKLKSTKEEP

SEQ ID NO: 375 - protein, 557 aa, synthetic construct
  source 1..557: note = Engineered CWCas12f1 (Q225T)
MGEKSSRRRRNGKSGAWTAAITSCVGGKMAKNTITKTLKLRIVRPYNSAEVEKIVADEKNNREKIALEKNKDKVKEACSKHLKVAAYCTTQVERNACLFCKARKLDDKFYQKLRGQFPDAVFWQEISEIFRQLQKQAAEIYNQSLIELYYEIFIKGKGIANASSVEHYLSDVCYTRAAELFKNAAIASGLRSKIKSNFRLKELKNMKSGLPTTKSDNFPIPLVKTKGGQYTGFEISNHNSDFIIKIPFGRWQVKKEIDKYRPWEKFDFEQVQKSPKPISLLLSTQRRKRNKGWSKDEGTEAEIKKVMNGDYQTSYIEVKRGSKIGEKSAWMLNLSIDVPKIDKGVDPSIIGGIDVGVKSPLVCAINNAFSRYSISDNDLFHFNKKMFARRRILLKKNRHKRAGHGAKNKLKPITILTEKSERFRKKLIERWACEIADFFIKNKVGTVQMENLESMKRKEDSYFNIRLRGFWPYAEMQNKIEFKLKQYGIEIRKVAPNNTSKTCSKCGHLNNYFNFEYRKKNKFPHFKCEKCNFKENADYNAALNISNPKLKSTKEEP

SEQ ID NO: 376 - protein, 557 aa, synthetic construct
  source 1..557: note = Engineered CWCas12f1 (Q225F)
MGEKSSRRRRNGKSGAWTAAITSCVGGKMAKNTITKTLKLRIVRPYNSAEVEKIVADEKNNREKIALEKNKDKVKEACSKHLKVAAYCTTQVERNACLFCKARKLDDKFYQKLRGQFPDAVFWQEISEIFRQLQKQAAEIYNQSLIELYYEIFIKGKGIANASSVEHYLSDVCYTRAAELFKNAAIASGLRSKIKSNFRLKELKNMKSGLPTTKSDNFPIPLVKFKGGQYTGFEISNHNSDFIIKIPFGRWQVKKEIDKYRPWEKFDFEQVQKSPKPISLLLSTQRRKRNKGWSKDEGTEAEIKKVMNGDYQTSYIEVKRGSKIGEKSAWMLNLSIDVPKIDKGVDPSIIGGIDVGVKSPLVCAINNAFSRYSISDNDLFHFNKKMFARRRILLKKNRHKRAGHGAKNKLKPITILTEKSERFRKKLIERWACEIADFFIKNKVGTVQMENLESMKRKEDSYFNIRLRGFWPYAEMQNKIEFKLKQYGIEIRKVAPNNTSKTCSKCGHLNNYFNFEYRKKNKFPHFKCEKCNFKENADYNAALNISNPKLKSTKEEP

SEQ ID NO: 377 - protein, 557 aa, synthetic construct
  source 1..557: note = Engineered CWCas12f1 (Q272K)
MGEKSSRRRRNGKSGAWTAAITSCVGGKMAKNTITKTLKLRIVRPYNSAEVEKIVADEKNNREKIALEKNKDKVKEACSKHLKVAAYCTTQVERNACLFCKARKLDDKFYQKLRGQFPDAVFWQEISEIFRQLQKQAAEIYNQSLIELYYEIFIKGKGIANASSVEHYLSDVCYTRAAELFKNAAIASGLRSKIKSNFRLKELKNMKSGLPTTKSDNFPIPLVKQKGGQYTGFEISNHNSDFIIKIPFGRWQVKKEIDKYRPWEKFDFEQVKKSPKPISLLLSTQRRKRNKGWSKDEGTEAEIKKVMNGDYQTSYIEVKRGSKIGEKSAWMLNLSIDVPKIDKGVDPSIIGGIDVGVKSPLVCAINNAFSRYSISDNDLFHFNKKMFARRRILLKKNRHKRAGHGAKNKLKPITILTEKSERFRKKLIERWACEIADFFIKNKVGTVQMENLESMKRKEDSYFNIRLRGFWPYAEMQNKIEFKLKQYGIEIRKVAPNNTSKTCSKCGHLNNYFNFEYRKKNKFPHFKCEKCNFKENADYNAALNISNPKLKSTKEEP

SEQ ID NO: 378 - protein, 249 aa, synthetic construct
  source 1..249: note = N-term 249aa extension
MVSKGEELFTGVVPILVELDGDVNGHKFSVSGEGEGDATYGKLTLKFICTTGKLPVPWPTLVTTLTYGVQCFSRYPDHMKQHDFFKSAMPEGYVQERTIFFKDDGNYKTRAEVKFEGDTLVNRIELKGIDFKEDGNILGHKLEYNYNSHNVYIMADKQKNGIKVNFKIRHNIEDGSVQLADHYQQNTPIGDGPVLLPDNHYLSTQSALSKDPNEKRDHMVLLEFVTAAGITLGMDELYKSGLRSRAQAL

SEQ ID NO: 379 - protein, 248 aa, synthetic construct
  source 1..248: note = C-term 248aa extension
RARDPPVATMVSKGEELFTGVVPILVELDGDVNGHKFSVSGEGEGDATYGKLTLKFICTTGKLPVPWPTLVTTLTYGVQCFSRYPDHMKQHDFFKSAMPEGYVQERTIFFKDDGNYKTRAEVKFEGDTLVNRIELKGIDFKEDGNILGHKLEYNYNSHNVYIMADKQKNGIKVNFKIRHNIEDGSVQLADHYQQNTPIGDGPVLLPDNHYLSTQSALSKDPNEKRDHMVLLEFVTAAGITLGMDELYK

SEQ ID NO: 380 - protein, 7 aa, synthetic construct
  source 1..7: note = Nuclear Localization Sequence
PKKKRKV

SEQ ID NO: 381 - protein, 16 aa, synthetic construct
  source 1..16: note = Nuclear Localization Sequence
KRPAATKKAGQAKKKK

SEQ ID NO: 382 - protein, 9 aa, synthetic construct
  source 1..9: note = Nuclear Localization Sequence
PAAKRVKLD

SEQ ID NO: 383 - protein, 11 aa, synthetic construct
  source 1..11: note = Nuclear Localization Sequence
RQRRNELKRSP

SEQ ID NO: 384 - protein, 38 aa, synthetic construct
  source 1..38: note = Nuclear Localization Sequence
NQSSNFGPMKGGNFGGRSSGPYGGGGQYFAKPRNQGGY

SEQ ID NO: 385 - protein, 42 aa, synthetic construct
  source 1..42: note = Nuclear Localization Sequence
RMRIZFKNKGKDTAELRRRRVEVSVELRKAKKDEQILKRRNV

SEQ ID NO: 386 - protein, 8 aa, synthetic construct
  source 1..8: note = Nuclear Localization Sequence
VSRKRPRP

SEQ ID NO: 387 - protein, 8 aa, synthetic construct
  source 1..8: note = Nuclear Localization Sequence
PPKKARED

SEQ ID NO: 388 - protein, 8 aa, synthetic construct
  source 1..8: note = Nuclear Localization Sequence
PQPKKKPL

SEQ ID NO: 389 - protein, 12 aa, synthetic construct
  source 1..12: note = Nuclear Localization Sequence
SALIKKKKKMAP

SEQ ID NO: 390 - protein, 5 aa, synthetic construct
  source 1..5: note = Nuclear Localization Sequence
DRLRR

SEQ ID NO: 391 - protein, 7 aa, synthetic construct
  source 1..7: note = Nuclear Localization Sequence
PKQKKRK

SEQ ID NO: 392 - protein, 10 aa, synthetic construct
  source 1..10: note = Nuclear Localization Sequence
RKLKKKIKKL

SEQ ID NO: 393 - protein, 10 aa, synthetic construct
  source 1..10: note = Nuclear Localization Sequence
REKKKFLKRR

SEQ ID NO: 394 - protein, 20 aa, synthetic construct
  source 1..20: note = Nuclear Localization Sequence
KRKGDEVDGVDEVAKKKSKK

SEQ ID NO: 395 - protein, 17 aa, synthetic construct
  source 1..17: note = Nuclear Localization Sequence
RKCLQAGMNLEARKTKK

SEQ ID NO: 396 - protein, 560 aa, synthetic construct
  source 1..560: note = Un1Cas12f1 with NLS
PKKKRKVGIHGVPAAMAKNTITKTLKLRIVRPYNSAEVEKIVADEKNNREKIALEKNKDKVKEACSKHLKVAAYCTTQVERNACLFCKARKLDDKFYQKLRGQFPDAVFWQEISEIFRQLQKQAAEIYNQSLIELYYEIFIKGKGIANASSVEHYLSDVCYTRAAELFKNAAIASGLRSKIKSNFRLKELKNMKSGLPTTKSDNFPIPLVKQKGGQYTGFEISNHNSDFIIKIPFGRWQVKKEIDKYRPWEKFDFEQVQKSPKPISLLLSTQRRKRNKGWSKDEGTEAEIKKVMNGDYQTSYIEVKRGSKIGEKSAWMLNLSIDVPKIDKGVDPSIIGGIDVGVKSPLVCAINNAFSRYSISDNDLFHFNKKMFARRRILLKKNRHKRAGHGAKNKLKPITILTEKSERFRKKLIERWACEIADFFIKNKVGTVQMENLESMKRKEDSYFNIRLRGFWPYAEMQNKIEFKLKQYGIEIRKVAPNNTSKTCSKCGHLNNYFNFEYRKKNKFPHFKCEKCNFKENADYNAALNISNPKLKSTKEEPKRPAATKKAGQAKKKK

SEQ ID NO: 397 - DNA, 20 bp, Homo sapiens
  source 1..20: mol_type = genomic DNA; note = PS-USH2A-F02
tgtctcgtctatcttgaatg

SEQ ID NO: 398 - DNA, 20 bp, Homo sapiens
  source 1..20: mol_type = genomic DNA; note = PS-USH2A-F03
tgttcgtatcatctgcagta

SEQ ID NO: 399 - DNA, 20 bp, Homo sapiens
  source 1..20: mol_type = genomic DNA; note = PS-USH2A-F05
agagtaagattggcccccta

SEQ ID NO: 400 - DNA, 20 bp, Homo sapiens
  source 1..20: mol_type = genomic DNA; note = PS-USH2A-F06
atttagctttaatatacaac

SEQ ID NO: 401 - DNA, 20 bp, Homo sapiens
  source 1..20: mol_type = genomic DNA; note = PS-USH2A-F07
atatacaactgtttgcgatg

SEQ ID NO: 402 - DNA, 20 bp, Homo sapiens
  source 1..20: mol_type = genomic DNA; note = PS-USH2A-F09
ttaaagagaaaaagagctcc

SEQ ID NO: 403 - DNA, 20 bp, Homo sapiens
  source 1..20: mol_type = genomic DNA; note = PS-USH2A-F10
aatgagcacatttgttaaaa

SEQ ID NO: 404 - DNA, 20 bp, Homo sapiens
  source 1..20: mol_type = genomic DNA; note = PS-USH2A-F12
ataaaaggttaagctgagta

SEQ ID NO: 405 - DNA, 22 bp, Homo sapiens
  source 1..22: mol_type = genomic DNA; note = PS-USH2A-F13
tactcagcttaaccttttatta

SEQ ID NO: 406 - DNA, 20 bp, Homo sapiens
  source 1..20: mol_type = genomic DNA; note = PS-USH2A-F15
gggtgagaacatttaagatc

SEQ ID NO: 407 - DNA, 20 bp, Homo sapiens
  source 1..20: mol_type = genomic DNA; note = PS-USH2A-F16
taatgtgtacatatatcaaa

SEQ ID NO: 408 - DNA, 20 bp, Homo sapiens
  source 1..20: mol_type = genomic DNA; note = PS-USH2A-F17
attataccttcgtgaagctg

SEQ ID NO: 409 - DNA, 20 bp, Homo sapiens
  source 1..20: mol_type = genomic DNA; note = PS-USH2A-F22
tattacttctatttaaagga

SEQ ID NO: 410 - DNA, 20 bp, Homo sapiens
  source 1..20: mol_type = genomic DNA; note = PS-USH2A-F23
gaataaccttacttgtcaga

SEQ ID NO: 411 - DNA, 20 bp, Homo sapiens
  source 1..20: mol_type = genomic DNA; note = PS-USH2A-F24
tttctttgccttgtaatacc

SEQ ID NO: 412 - DNA, 20 bp, Homo sapiens
  source 1..20: mol_type = genomic DNA; note = PS-USH2A-F25
catctaaacatttactattc

SEQ ID NO: 413 - DNA, 20 bp, Homo sapiens
  source 1..20: mol_type = genomic DNA; note = PS-USH2A-F26
gatgcaaaatacttccttta

SEQ ID NO: 414 - DNA, 20 bp, Homo sapiens
  source 1..20: mol_type = genomic DNA; note = PS-USH2A-F27
gaaactatctaaaggaagta

SEQ ID NO: 415 - DNA, 20 bp, Homo sapiens
  source 1..20: mol_type = genomic DNA; note = PS-USH2A-F30
aattgcaattatagcttgaa

SEQ ID NO: 416 - DNA, 21 bp, Homo sapiens
  source 1..21: mol_type = genomic DNA; note = PS-USH2A-FA01
aaaggtgaggatgggaaaatg

SEQ ID NO: 417 - DNA, 22 bp, Homo sapiens
  source 1..22: mol_type = genomic DNA; note = PS-USH2A-FA02
tgaagttcatcgcaaacagttg

SEQ ID NO: 418 - DNA, 20 bp, Homo sapiens
  source 1..20: mol_type = genomic DNA; note = PS-USH2A-FA03
attattacttaatgcaaaga

SEQ ID NO: 419 - DNA, 20 bp, Homo sapiens
  source 1..20: mol_type = genomic DNA; note = PS-USH2A-FA04
cattaagtaataattaaaaa

SEQ ID NO: 420 - DNA, 21 bp, Homo sapiens
  source 1..21: mol_type = genomic DNA; note = PS-USH2A-FA05
aaattatagtagaattacata

SEQ ID NO: 421 - DNA, 19 bp, Homo sapiens
  source 1..19: mol_type = genomic DNA; note = PS-USH2A-FA06
agatctaatctcttagcaa

SEQ ID NO: 422 - DNA, 20 bp, Homo sapiens
  source 1..20: mol_type = genomic DNA; note = PS-USH2A-FA07
atatatgtacacattataaa

SEQ ID NO: 423 - DNA, 22 bp, Homo sapiens
  source 1..22: mol_type = genomic DNA; note = PS-USH2A-FA08
tggcagacaacatgatgttttg

SEQ ID NO: 424 - DNA, 21 bp, Homo sapiens
  source 1..21: mol_type = genomic DNA; note = PS-USH2A-FA09
tttaattataccttcgtgaag

SEQ ID NO: 425 - DNA, 20 bp, Homo sapiens
  source 1..20: mol_type = genomic DNA; note = PS-USH2A-FA10
acagtgatgaatgactcacc

SEQ ID NO: 426 - DNA, 20 bp, Homo sapiens
  source 1..20: mol_type = genomic DNA; note = PS-USH2A-FA11
atttcaataaggaaaataaa

SEQ ID NO: 427 - DNA, 20 bp, Homo sapiens
  source 1..20: mol_type = genomic DNA; note = PS-USH2A-FA12
tccatatatatacatatata

SEQ ID NO: 428 - DNA, 21 bp, Homo sapiens
  source 1..21: mol_type = genomic DNA; note = PS-USH2A-FA13
ggaaatgcttttctacatatg

SEQ ID NO: 429 - DNA, 20 bp, Homo sapiens
  source 1..20: mol_type = genomic DNA; note = PS-USH2A-FA14
ttttccttattgaaattaaa

SEQ ID NO: 430 - DNA, 20 bp, Homo sapiens
  source 1..20: mol_type = genomic DNA; note = PS-USH2A-FA15
aaaataactgtattgttaac

SEQ ID NO: 431 - DNA, 20 bp, Homo sapiens
  source 1..20: mol_type = genomic DNA; note = PS-USH2A-FA16
aactattaaaattggtctac

SEQ ID NO: 432 - DNA, 20 bp, Homo sapiens
  source 1..20: mol_type = genomic DNA; note = PS-USH2A-FA17
aaactgatatgatatgaatc

SEQ ID NO: 433 - DNA, 20 bp, Homo sapiens
  source 1..20: mol_type = genomic DNA; note = PS-USH2A-FA18
atagttcaaaatgagtcata

SEQ ID NO: 434 - DNA, 19 bp, Homo sapiens
  source 1..19: mol_type = genomic DNA; note = PS-USH2A-FA19
aaatttgcagcaatagtgg

SEQ ID NO: 435 - DNA, 19 bp, Homo sapiens
  source 1..19: mol_type = genomic DNA; note = PS-USH2A-FA20
aatatgccatacatattcc

SEQ ID NO: 436 - DNA, 19 bp, Homo sapiens
  source 1..19: mol_type = genomic DNA; note = PS-USH2A-FA21
aaaatatgcacagtgctta

SEQ ID NO: 437 - DNA, 20 bp, Homo sapiens
  source 1..20: mol_type = genomic DNA; note = PS-USH2A-FA22
aaaattaatcttaaaataag

SEQ ID NO: 438 - DNA, 20 bp, Homo sapiens
  source 1..20: mol_type = genomic DNA; note = PS-USH2A-FA23
aattcatggatatttggaaa

SEQ ID NO: 439 - DNA, 21 bp, Homo sapiens
  source 1..21: mol_type = genomic DNA; note = PS-USH2A-FA24
tcacctaaacttaaatctctg

SEQ ID NO: 440 - DNA, 20 bp, Homo sapiens
  source 1..20: mol_type = genomic DNA; note = PS-USH2A-FA25
aagaggtatgttctgagtca

SEQ ID NO: 441 - DNA, 20 bp, Homo sapiens
  source 1..20: mol_type = genomic DNA; note = PS-USH2A-FA26
tattaattgaaaatgataaa

SEQ ID NO: 442 - DNA, 20 bp, Homo sapiens
  source 1..20: mol_type = genomic DNA; note = PS-USH2A-FA27
tatgctcctctattttatca

SEQ ID NO: 443 - DNA, 20 bp, Homo sapiens
  source 1..20: mol_type = genomic DNA; note = PS-USH2A-FA28
agtaattaatataaataaaa

SEQ ID NO: 444 - DNA, 21 bp, Homo sapiens
  source 1..21: mol_type = genomic DNA; note = PS-USH2A-FA29
tgaaaacagcatatacactta

SEQ ID NO: 445 - DNA, 21 bp, Homo sapiens
  source 1..21: mol_type = genomic DNA; note = PS-USH2A-FA30
gatagtttccaaatatccatg

SEQ ID NO: 446 - DNA, 20 bp, Homo sapiens
  source 1..20: mol_type = genomic DNA; note = PS-USH2A-R01
ttaacttaggtaacttctcc

SEQ ID NO: 447 - DNA, 20 bp, Homo sapiens
  source 1..20: mol_type = genomic DNA; note = PS-USH2A-R02
gaaataaaatttgtagaagc

SEQ ID NO: 448 - DNA, 20 bp, Homo sapiens
  source 1..20: mol_type = genomic DNA; note = PS-USH2A-R04
gataaaactcagccgatcgg

SEQ ID NO: 449 - DNA, 20 bp, Homo sapiens
  source 1..20: mol_type = genomic DNA; note = PS-USH2A-R05
cttcaagtgtagaaattgag

SEQ ID NO: 450 - DNA, 20 bp, Homo sapiens
  source 1..20: mol_type = genomic DNA; note = PS-USH2A-R07
agttgaatatccatacaatg

SEQ ID NO: 451 - DNA, 20 bp, Homo sapiens
  source 1..20: mol_type = genomic DNA; note = PS-USH2A-R08
gcattgtatggatattcaac

SEQ ID NO: 452 - DNA, 20 bp, Homo sapiens
  source 1..20: mol_type = genomic DNA; note = PS-USH2A-R09
ttcagagatttagttcatca

SEQ ID NO: 453 - DNA, 20 bp, Homo sapiens
  source 1..20: mol_type = genomic DNA; note = PS-USH2A-R10
tatagaaatacctagaattg

SEQ ID NO: 454 - DNA, 20 bp, Homo sapiens
  source 1..20: mol_type = genomic DNA; note = PS-USH2A-R11
atggcatgtggaaacaattc

SEQ ID NO: 455 - DNA, 20 bp, Homo sapiens
  source 1..20: mol_type = genomic DNA; note = PS-USH2A-R13
ttaatttgatggcatgtgga

SEQ ID NO: 456 - DNA, 20 bp, Homo sapiens
  source 1..20: mol_type = genomic DNA; note = PS-USH2A-R14
tatataatgagattaaacag

SEQ ID NO: 457 - DNA, 20 bp, Homo sapiens
  source 1..20: mol_type = genomic DNA; note = PS-USH2A-R17
gttaaaatcttaaatgtaag

SEQ ID NO: 458 - DNA, 20 bp, Homo sapiens
  source 1..20: mol_type = genomic DNA; note = PS-USH2A-R18
tagacccatataactcagag

SEQ ID NO: 459 - DNA, 20 bp, Homo sapiens
  source 1..20: mol_type = genomic DNA; note = PS-USH2A-R19
cttgccagagaaggagtaga

SEQ ID NO: 460 - DNA, 20 bp, Homo sapiens
  source 1..20: mol_type = genomic DNA; note = PS-USH2A-R20
ttctactccttctctggcaa

SEQ ID NO: 461 - DNA, 20 bp, Homo sapiens
  source 1..20: mol_type = genomic DNA; note = PS-USH2A-R22
gcattggtcagtgtgtaaga

SEQ ID NO: 462 - DNA, 20 bp, Homo sapiens
  source 1..20: mol_type = genomic DNA; note = PS-USH2A-R23
atacttacatcacaaaaaga

SEQ ID NO: 463 - DNA, 20 bp, Homo sapiens
  source 1..20: mol_type = genomic DNA; note = PS-USH2A-R24
tggagtatctagttataata

SEQ ID NO: 464 - DNA, 20 bp, Homo sapiens
  source 1..20: mol_type = genomic DNA; note = PS-USH2A-R26
taattctaccaccagccaca

SEQ ID NO: 465 - DNA, 20 bp, Homo sapiens
  source 1..20: mol_type = genomic DNA; note = PS-USH2A-R27
ttagctacctcttagttata

SEQ ID NO: 466 - DNA, 20 bp, Homo sapiens
  source 1..20: mol_type = genomic DNA; note = PS-USH2A-R29
tttggttggttacctctgag

SEQ ID NO: 467 - DNA, 20 bp, Homo sapiens
  source 1..20: mol_type = genomic DNA; note = PS-USH2A-R30
gttggttacctctgagccaa

SEQ ID NO: 468 - DNA, 20 bp, Homo sapiens
  source 1..20: mol_type = genomic DNA; note = PS-USH2A-R31
taagtacgtgacacccctgg

SEQ ID NO: 469 - DNA, 20 bp, Homo sapiens
  source 1..20: mol_type = genomic DNA; note = PS-USH2A-R32
gggaccatttcatcaggtag

SEQ ID NO: 470 - DNA, 20 bp, Homo sapiens
  source 1..20: mol_type = genomic DNA; note = PS-USH2A-R34
ccttcaggttaatcctttca

SEQ ID NO: 471 - DNA, 20 bp, Homo sapiens
  source 1..20: mol_type = genomic DNA; note = PS-USH2A-R35
gcaacaaagtcctttgtctc

SEQ ID NO: 472 - DNA, 20 bp, Homo sapiens
  source 1..20: mol_type = genomic DNA; note = PS-USH2A-R36
actgtgtaggagacaaagga

SEQ ID NO: 473 - DNA, 20 bp, Homo sapiens
  source 1..20: mol_type = genomic DNA; note = PS-USH2A-R38
tacacctaccagatatctaa

SEQ ID NO: 474 - DNA, 20 bp, Homo sapiens
  source 1..20: mol_type = genomic DNA; note = PS-USH2A-R39
atctacaccatgcataagac

SEQ ID NO: 475 - DNA, 20 bp, Homo sapiens
  source 1..20: mol_type = genomic DNA; note = PS-USH2A-R40
cttagaaagaaggatgtata

SEQ ID NO: 476 - DNA, 26 bp, synthetic construct
  source 1..26: mol_type = other DNA; note = USH2A-F-F#1
aggattaaaccaaaaattgccctgga

SEQ ID NO: 477 - DNA, 26 bp, synthetic construct
  source 1..26: mol_type = other DNA; note = USH2A-F-F#2
caccatgctgtacaatagagctccag

SEQ ID NO: 478 - DNA, 26 bp, synthetic construct
  source 1..26: mol_type = other DNA; note = USH2A-F-F#3
ggcattgcttgtgagaaaacactcaa

SEQ ID NO: 479 - DNA, 27 bp, synthetic construct
  source 1..27: mol_type = other DNA; note = USH2A-F-F#4
agagctccagcatatgtaacagaaaca

SEQ ID NO: 480 - DNA, 26 bp, synthetic construct
  source 1..26: mol_type = other DNA; note = USH2A-F-F#7
tgccttaggtgagtcattcatcactg

SEQ ID NO: 481 - DNA, 28 bp, synthetic construct
  source 1..28: mol_type = other DNA; note = USH2A-F-F#8
agaacttgccttcattggagttcttgaa

SEQ ID NO: 482 - DNA, 26 bp, synthetic construct
  source 1..26: mol_type = other DNA; note = USH2A-F-F#10
tgagttcctgagtatgtttttgactc

SEQ ID NO: 483 - DNA, 26 bp, synthetic construct
  source 1..26: mol_type = other DNA; note = USH2A-F-R#1
tttgttcactgagccatggaggttac

SEQ ID NO: 484 - DNA, 26 bp, synthetic construct
  source 1..26: mol_type = other DNA; note = USH2A-F-R#3
tgtttctgttacatatgctggagctc

SEQ ID NO: 485 - DNA, 26 bp, synthetic construct
  source 1..26: mol_type = other DNA; note = USH2A-F-R#4
aatttgttcactgagccatggaggtt

SEQ ID NO: 486 - DNA, 26 bp, synthetic construct
  source 1..26: mol_type = other DNA; note = USH2A-F-R#8
tccagggcaatttttggtttaatcct

SEQ ID NO: 487 - DNA, 26 bp, synthetic construct
  source 1..26: mol_type = other DNA; note = USH2A-R-F#1
gagtgtgattccttggggacattacc

SEQ ID NO: 488 - DNA, 26 bp, synthetic construct
  source 1..26: mol_type = other DNA; note = USH2A-R-F#3
tggctaaatgtttttgctgaagaggc

SEQ ID NO: 489 - DNA, 26 bp, synthetic construct
  source 1..26: mol_type = other DNA; note = USH2A-R-F#4
aaactcagccgatcggatttatttca

SEQ ID NO: 490 - DNA, 28 bp, synthetic construct
  source 1..28: mol_type = other DNA; note = USH2A-R-F#8
agcaaagaatccagcctaggataattgg

SEQ ID NO: 491 - DNA, 28 bp, synthetic construct
  source 1..28: mol_type = other DNA; note = USH2A-R-F#9
ccaggggtgtcacgtacttataaaatga

SEQ ID NO: 492 - DNA, 28 bp, synthetic construct
  source 1..28: mol_type = other DNA; note = USH2A-R-F#10
caaagtcctttgtctcctacacagtcaa

SEQ ID NO: 493 - DNA, 26 bp, synthetic construct
  source 1..26: mol_type = other DNA; note = USH2A-R-R#1
tacacactgaccaatgccaaaggaaa

SEQ ID NO: 494 - DNA, 26 bp, synthetic construct
  source 1..26: mol_type = other DNA; note = USH2A-R-R#2
gcctcttcagcaaaaacatttagcca

SEQ ID NO: 495 - DNA, 26 bp, synthetic construct
  source 1..26: mol_type = other DNA; note = USH2A-R-R#3
attggctgacaggacaacaattagca

SEQ ID NO: 496 - DNA, 28 bp, synthetic construct
  source 1..28: mol_type = other DNA; note = USH2A-R-R#8
tcttcctgtcttctgggatacttaccac

SEQ ID NO: 497 - DNA, 28 bp, synthetic construct
  source 1..28: mol_type = other DNA; note = USH2A-R-R#9
ggaccaaagggaacaaatgtttgtaact

SEQ ID NO: 498 - DNA, 28 bp, synthetic construct
  source 1..28: mol_type = other DNA; note = USH2A-R-R#10
gagagccacaaagataaaggaaagagca

SEQ ID NO: 499 - DNA, 26 bp, synthetic construct
  source 1..26: mol_type = other DNA; note = USH2A-R-R#11
ttctaattcctgagtcctgactgcag

SEQ ID NO: 500 - DNA, 58 bp, synthetic construct
  source 1..58: mol_type = other DNA; note = USH2A-F-F#1 miseq F
cactctttccctacacgacgctcttccgatctaggattaaaccaaaaattgccctgga

SEQ ID NO: 501 - DNA, 58 bp, synthetic construct
  source 1..58: mol_type = other DNA; note = USH2A-F-F#2 miseq F
cactctttccctacacgacgctcttccgatctcaccatgctgtacaatagagctccag

SEQ ID NO: 502 - DNA, 58 bp, synthetic construct
  source 1..58: mol_type = other DNA; note = USH2A-F-F#3 miseq F
cactctttccctacacgacgctcttccgatctggcattgcttgtgagaaaacactcaa

SEQ ID NO: 503 - DNA, 59 bp, synthetic construct
  source 1..59: mol_type = other DNA; note = USH2A-F-F#4 miseq F
cactctttccctacacgacgctcttccgatctagagctccagcatatgtaacagaaaca

SEQ ID NO: 504 - DNA, 58 bp, synthetic construct
  source 1..58: mol_type = other DNA; note = USH2A-F-F#5 miseq F
cactctttccctacacgacgctcttccgatctctgaaactttgtactcagcttaacct

SEQ ID NO: 505 - DNA, 60 bp, synthetic construct
  source 1..60: mol_type = other DNA; note = USH2A-F-F#6 miseq F
cactctttccctacacgacgctcttccgatcttttttcccagcttcacgaaggtataatt

SEQ ID NO: 506 - DNA, 57 bp, synthetic construct
  source 1..57: mol_type = other DNA; note = USH2A-F-F#9 miseq F
cactctttccctacacgacgctcttccgatctctttgccttgtaatacccttttatc

SEQ ID NO: 507 - DNA, 58 bp, synthetic construct
  source 1..58: mol_type = other DNA; note = USH2A-F-F#10 miseq F
cactctttccctacacgacgctcttccgatcttgagttcctgagtatgtttttgactc

SEQ ID NO: 508 - DNA, 60 bp, synthetic construct
  source 1..60: mol_type = other DNA; note = USH2A-F-R#3 miseq R
gtgactggagttcagacgtgtgctcttccgatcttgtttctgttacatatgctggagctc

SEQ ID NO: 509 - DNA, 60 bp, synthetic construct
  source 1..60: mol_type = other DNA; note = USH2A-F-R#4 miseq R
gtgactggagttcagacgtgtgctcttccgatctaatttgttcactgagccatggaggtt

SEQ ID NO: 510 - DNA, 60 bp, synthetic construct
  source 1..60: mol_type = other DNA; note = USH2A-F-R#5 miseq R
gtgactggagttcagacgtgtgctcttccgatctagacgagacacaaacaatgctactgc

SEQ ID NO: 511 - DNA, 59 bp, synthetic construct
  source 1..59: mol_type = other DNA; note = USH2A-F-R#6 miseq R
gtgactggagttcagacgtgtgctcttccgatctcaactgtttgcgatgaacttcataa

SEQ ID NO: 512 - DNA, 60 bp, synthetic construct
  source 1..60: mol_type = other DNA; note = USH2A-F-R#7 miseq R
gtgactggagttcagacgtgtgctcttccgatctctggagctctattgtacagcatggtg

SEQ ID NO: 513 - DNA, 60 bp, synthetic construct
  source 1..60: mol_type = other DNA; note = USH2A-F-R#9 miseq R
gtgactggagttcagacgtgtgctcttccgatctcattgcttgtcatcttgtgtgactca

SEQ ID NO: 514 - DNA, 65 bp, synthetic construct
  source 1..65: mol_type = other DNA; note = USH2A-F-R#10 miseq R
gtgactggagttcagacgtgtgctcttccgatctcacctaaacttaaatctctgacaagtaaggt

SEQ ID NO: 515 - DNA, 65 bp, synthetic construct
  source 1..65: mol_type = other DNA; note = USH2A-F-R#11 miseq R
gtgactggagttcagacgtgtgctcttccgatctgtacatatatcaaaacatcatgttgtctgcc

SEQ ID NO: 516 - DNA, 58 bp, synthetic construct
  source 1..58: mol_type = other DNA; note = USH2A-R-F#2 miseq F
cactctttccctacacgacgctcttccgatctacattttcagtgcacaatgacattcc

SEQ ID NO: 517 - DNA, 58 bp, synthetic construct
  source 1..58: mol_type = other DNA; note = USH2A-R-F#3 miseq F
cactctttccctacacgacgctcttccgatcttggctaaatgtttttgctgaagaggc

SEQ ID NO: 518 - DNA, 58 bp, synthetic construct
  source 1..58: mol_type = other DNA; note = USH2A-R-F#4 miseq F
cactctttccctacacgacgctcttccgatctaaactcagccgatcggatttatttca

SEQ ID NO: 519 - DNA, 58 bp, synthetic construct
  source 1..58: mol_type = other DNA; note = USH2A-R-F#5 miseq F
cactctttccctacacgacgctcttccgatctaacttctccctgtttctggtttgtgg

SEQ ID NO: 520 - DNA, 59 bp, synthetic construct
  source 1..59: mol_type = other DNA; note = USH2A-R-F#6 miseq F
cactctttccctacacgacgctcttccgatctacctagaattgtttccacatgccatca

SEQ ID NO: 521 - DNA, 58 bp, synthetic construct
  source 1..58: mol_type = other DNA; note = USH2A-R-F#7 miseq F
cactctttccctacacgacgctcttccgatctgaccccatctatggctctccttacat

SEQ ID NO: 522 - DNA, 60 bp, synthetic construct
  source 1..60: mol_type = other DNA; note = USH2A-R-F#8 miseq F
cactctttccctacacgacgctcttccgatctagcaaagaatccagcctaggataattgg

SEQ ID NO: 523 - DNA, 60 bp, synthetic construct
  source 1..60: mol_type = other DNA; note = USH2A-R-F#9 miseq F
cactctttccctacacgacgctcttccgatctccaggggtgtcacgtacttataaaatga

SEQ ID NO: 524 - DNA, 58 bp, synthetic construct
  source 1..58: mol_type = other DNA; note = USH2A-R-F#11 miseq F
cactctttccctacacgacgctcttccgatctctaggataattgggccatgcttttcc

SEQ ID NO: 525 - DNA, 58 bp, synthetic construct
  source 1..58: mol_type = other DNA; note = USH2A-R-F#12 miseq F
cactctttccctacacgacgctcttccgatctataattctaccaccagccacaacaga

SEQ ID NO: 526 - DNA, 56 bp, synthetic construct
  source 1..56: mol_type = other DNA; note = USH2A-R-F#13 miseq F
cactctttccctacacgacgctcttccgatcttttggcaacaaagtcctttgtctc

SEQ ID NO: 527 - DNA, 58 bp, synthetic construct
  source 1..58: mol_type = other DNA; note = USH2A-R-F#14 miseq F
cactctttccctacacgacgctcttccgatctcttatccgttgtttaacagctgtgct

SEQ ID NO: 528 - DNA, 58 bp, synthetic construct
  source 1..58: mol_type = other DNA; note = USH2A-R-F#15 miseq F
cactctttccctacacgacgctcttccgatcttttctctacatgggtatatggccacc

SEQ ID NO: 529 - DNA, 58 bp, synthetic construct
  source 1..58: mol_type = other DNA; note = USH2A-R-F#16 miseq F
cactctttccctacacgacgctcttccgatcttcatcaggtagaagcaaggtggtaag

SEQ ID NO: 530 - DNA, 58 bp, synthetic construct
  source 1..58: mol_type = other DNA; note = USH2A-R-F#17 miseq F
cactctttccctacacgacgctcttccgatctacagcctaaatgacagatacagcaca

SEQ ID NO: 531 - DNA, 58 bp, synthetic construct
  source 1..58: mol_type = other DNA; note = USH2A-R-F#18 miseq F
cactctttccctacacgacgctcttccgatcttccttccaatgaaagacccaatccat

SEQ ID NO: 532 - DNA, 60 bp, synthetic construct
  source 1..60: mol_type = other DNA; note = USH2A-R-R#1 miseq R
gtgactggagttcagacgtgtgctcttccgatcttacacactgaccaatgccaaaggaaa

SEQ ID NO: 533 - DNA, 60 bp, synthetic construct
  source 1..60: mol_type = other DNA; note = USH2A-R-R#2 miseq R
gtgactggagttcagacgtgtgctcttccgatctgcctcttcagcaaaaacatttagcca

SEQ ID NO: 534 - DNA, 60 bp, synthetic construct
  source 1..60: mol_type = other DNA; note = USH2A-R-R#4 miseq R
gtgactggagttcagacgtgtgctcttccgatcttgaaataaatccgatcggctgagttt

SEQ ID NO: 535 - DNA, 60 bp, synthetic construct
  source 1..60: mol_type = other DNA; note = USH2A-R-R#5 miseq R
gtgactggagttcagacgtgtgctcttccgatctaaatgtaaggagagccatagatgggg

SEQ ID NO: 536 - DNA, 60 bp, synthetic construct
  source 1..60: mol_type = other DNA; note = USH2A-R-R#6 miseq R
gtgactggagttcagacgtgtgctcttccgatctacaggacaacaattagcacagctgtt

SEQ ID NO: 537 - DNA, 60 bp, synthetic construct
  source 1..60: mol_type = other DNA; note = USH2A-R-R#7 miseq R
gtgactggagttcagacgtgtgctcttccgatcttactccttctctggcaagcaaatcac

SEQ ID NO: 538 - DNA, 62 bp, synthetic construct
  source 1..62: mol_type = other DNA; note = USH2A-R-R#10 miseq R
gtgactggagttcagacgtgtgctcttccgatctgagagccacaaagataaaggaaagagca

SEQ ID NO: 539 - DNA, 60 bp, synthetic construct
  source 1..60: mol_type = other DNA; note = USH2A-R-R#11 miseq R
gtgactggagttcagacgtgtgctcttccgatctttctaattcctgagtcctgactgcag

SEQ ID NO: 540 - DNA, 60 bp, synthetic construct
  source 1..60: mol_type = other DNA; note = USH2A-R-R#12 miseq R
gtgactggagttcagacgtgtgctcttccgatctcttaccaccttgcttctacctgatga

SEQ ID NO: 541 - DNA, 60 bp, synthetic construct
  source 1..60: mol_type = other DNA; note = USH2A-R-R#13 miseq R
gtgactggagttcagacgtgtgctcttccgatctggaaggaccaaagggaacaaatgttt

SEQ ID NO: 542 - DNA, 65 bp, synthetic construct
  source 1..65: mol_type = other DNA; note = USH2A-R-R#14 miseq R
gtgactggagttcagacgtgtgctcttccgatctggagatttacttcaagtgtagaaattgagtc

SEQ ID NO: 543 - DNA, 60 bp, synthetic construct
  source 1..60: mol_type = other DNA; note = USH2A-R-R#15 miseq R
gtgactggagttcagacgtgtgctcttccgatcttgtgctgtatctgtcatttaggctgt

SEQ ID NO: 544 - DNA, 60 bp, synthetic construct
  source 1..60: mol_type = other DNA; note = USH2A-R-R#16 miseq R
gtgactggagttcagacgtgtgctcttccgatctttgactgtgtaggagacaaaggactt

SEQ ID NO: 545 - DNA, 65 bp, synthetic construct
  source 1..65: mol_type = other DNA; note = USH2A-R-R#17 miseq R
gtgactggagttcagacgtgtgctcttccgatctgcttgttttggtttacttagaaagaaggatg